European Patent Application EP 4 122 948 A1, published January 25, 2023. Title: Synthetic polymer, Production method thereof, Molding material composition and Moldied article. Applicant: Spiber Inc. The sequence listing filed with the application follows.

SEQUENCE LISTING (72 sequences)

SEQ ID NO: 1 - protein, 50 aa, Araneus diadematus
SGCDVLVQALLEVVSALVSILGSSSIGQINYGASAQYTQMVGQSVAQALA

SEQ ID NO: 2 - protein, 30 aa, Araneus diadematus
SGCDVLVQALLEVVSALVSILGSSSIGQIN

SEQ ID NO: 3 - protein, 21 aa, Araneus diadematus
SGCDVLVQALLEVVSALVSIL

SEQ ID NO: 4 - protein, 1154 aa, Artificial Sequence
  recombinant spider silk protein ADF3KaiLargeNRSH1
MHHHHHHHHHHSSGSSLEVLFQGPARAGSGQQGPGQQGPGQQGPGQQGPYGPGASAAAAAAGGYGPGSGQQGPSQQGPGQQGPGGQGPYGPGASAAAAAAGGYGPGSGQQGPGGQGPYGPGSSAAAAAAGGNGPGSGQQGAGQQGPGQQGPGASAAAAAAGGYGPGSGQQGPGQQGPGGQGPYGPGASAAAAAAGGYGPGSGQGPGQQGPGGQGPYGPGASAAAAAAGGYGPGSGQQGPGQQGPGQQGPGGQGPYGPGASAAAAAAGGYGPGYGQQGPGQQGPGGQGPYGPGASAASAASGGYGPGSGQQGPGQQGPGGQGPYGPGASAAAAAAGGYGPGSGQQGPGQQGPGQQGPGQQGPGGQGPYGPGASAAAAAAGGYGPGSGQQGPGQQGPGQQGPGQQGPGQQGPGQQGPGQQGPGQQGPGQQGPGGQGAYGPGASAAAGAAGGYGPGSGQQGPGQQGPGQQGPGQQGPGQQGPGQQGPGQQGPGQQGPYGPGASAAAAAAGGYGPGSGQQGPGQQGPGQQGPGGQGPYGPGAASAAVSVSRARAGSGQQGPGQQGPGQQGPGQQGPYGPGASAAAAAAGGYGPGSGQQGPSQQGPGQQGPGGQGPYGPGASAAAAAAGGYGPGSGQQGPGGQGPYGPGSSAAAAAAGGNGPGSGQQGAGQQGPGQQGPGASAAAAAAGGYGPGSGQQGPGQQGPGGQGPYGPGASAAAAAAGGYGPGSGQGPGQQGPGGQGPYGPGASAAAAAAGGYGPGSGQQGPGQQGPGQQGPGGQGPYGPGASAAAAAAGGYGPGYGQQGPGQQGPGGQGPYGPGASAASAASGGYGPGSGQQGPGQQGPGGQGPYGPGASAAAAAAGGYGPGSGQQGPGQQGPGQQGPGQQGPGGQGPYGPGASAAAAAAGGYGPGSGQQGPGQQGPGQQGPGQQGPGQQGPGQQGPGQQGPGQQGPGQQGPGGQGAYGPGASAAAGAAGGYGPGSGQQGPGQQGPGQQGPGQQGPGQQGPGQQGPGQQGPGQQGPYGPGASAAAAAAGGYGPGSGQQGPGQQGPGQQGPGGQGPYGPGAASAAVSVGGYGPQSSSVPVASAVASRLSSPAASSRVSSAVSSLVSSGPTKHAALSNTISSVVSQVSASNPGLSGCDVLVQALLEVVSALVSIL

SEQ ID NO: 5 - protein, 24 aa, Artificial Sequence
  His tag and start codon
MHHHHHHHHHHSSGSSLEVLFQGP

SEQ ID NO: 6 - protein, 597 aa, Artificial Sequence
  Met-PRT380
MGPGQQGPYGPGASAAAAAGQNGPGSGQQGPGQSAAAAAGQYGPGQQGPGQQGPGSSAAAAAGPGQYGPGQQGPSASAAAAAGPGSGQQGPGASAAAAAGQYGPGQQGPGQQGPGSSAAAAAGQYGSGPGQQGPYGSAAAAAGPGSGQYGQGPYGPGASAAAAAGPGQYGPGQQGPSASAAAAAGSGQQGPGQYGPYASAAAAAGQYGSGPGQQGPYGPGQSAAAAAGSGQQGPGQQGPYASAAAAAGPGQQGPYGPGSSAAAAAGQYGYGPGQQGPYGPGASAAAAAGQNGPGSGQYGPGQQGPGQSAAAAAGPGQQGPYGPGASAAAAAGQYGPGQQGPGQYGPGSSAAAAAGPGQQGPYGPGSSAAAAAGQYGPGQQGPYGPGQSAAAAAGQYQQGPGQQGPYGPGASAAAAAGPGQQGPYGPGASAAAAAGPGQYGPGQQGPSASAAAAAGQYGSGPGQYGPYGPGQSAAAAAGPGSGQQGQGPYGPGASAAAAAGQYGPGQQGPYGPGQSAAAAAGPGSGQYGPGASAAAAAGQNGPGSGQYGPGQQGPGQSAAAAAGQYQQGPGQQGPYGPGASAAAAAGPGSGQQGPGAS

SEQ ID NO: 7 - protein, 590 aa, Artificial Sequence
  Met-PRT410
MGPGQQGPYGPGASAAAAAGQNGPGSGQQGPGQSGQYGPGQQGPGQQGPGSSAAAAAGPGQYGPGQQGPSASAAAAAGPGSGQQGPGASGQYGPGQQGPGQQGPGSSAAAAAGQYGSGPGQQGPYGSAAAAAGPGSGQYGQGPYGPGASGPGQYGPGQQGPSASAAAAAGSGQQGPGQYGPYASAAAAAGQYGSGPGQQGPYGPGQSGSGQQGPGQQGPYASAAAAAGPGQQGPYGPGSSAAAAAGQYGYGPGQQGPYGPGASGQNGPGSGQYGPGQQGPGQSAAAAAGPGQQGPYGPGASAAAAAGQYGPGQQGPGQYGPGSSGPGQQGPYGPGSSAAAAAGQYGPGQQGPYGPGQSAAAAAGQYQQGPGQQGPYGPGASGPGQQGPYGPGASAAAAAGPGQYGPGQQGPSASAAAAAGQYGSGPGQYGPYGPGQSGPGSGQQGQGPYGPGASAAAAAGQYGPGQQGPYGPGQSAAAAAGPGSGQYGPGASGQNGPGSGQYGPGQQGPGQSAAAAAGQYQQGPGQQGPYGPGASAAAAAGQYGSGPGQQGPYGPGQSGSGQQGPGQQGPYASAAAAAGPGSGQQGPGAS

SEQ ID NO: 8 - protein, 565 aa, Artificial Sequence
  Met-PRT525
MGPGQQGPYGPGASAAAAAAAGSNGPGSGQQGPGQSGQYGPGQQGPGQQGPGSSAAAAAAAGPGQYGPGQQGPSASAAAAAAAGPGSGQQGPGASGQYGPGQQGPGQQGPGSSAAAAAAAGSYGSGPGQQGPYGSAAAAAAAGPGSGQYGQGPYGPGASGPGQYGPGQQGPSASAAAAAAAGSGQQGPGQYGPYASAAAAAAAGSYGSGPGQQGPYGPGQSGSGQQGPGQQGPYASAAAAAAAGPGQQGPYGPGSSAAAAAAAGSYGYGPGQQGPYGPGASGQNGPGSGQYGPGQQGPGPSAAAAAAAGPGQQGPYGPGASAAAAAAAGSYGPGQQGPGQYGPGSSGPGQQGPYGPGSSAAAAAAAGSYGPGQQGPYGPGPSAAAAAAAGSYQQGPGQQGPYGPGASGPGQQGPYGPGASAAAAAAAGPGQYGPGQQGPSASAAAAAAAGSYGSGPGQYGPYGPGQSGPGSGQQGQGPYGPGASAAAAAAAGSYGPGQQGPYGPGPSAAAAAAAGPGSGQYGPGASGQNGPGSGQYGPGQQGPGPSAAAAAAAGPGSGQQGPGAS

SEQ ID NO: 9 - protein, 2364 aa, Artificial Sequence
  Met-PRT799
MGPGQQGPYGPGASAAAAAGQNGPGSGQQGPGQSGQYGPGQQGPGQQGPGSSAAAAAGPGQYGPGQQGPSASAAAAAGPGSGQQGPGASGQYGPGQQGPGQQGPGSSAAAAAGQYGSGPGQQGPYGSAAAAAGPGSGQYGQGPYGPGASGPGQYGPGQQGPSASAAAAAGSGQQGPGQYGPYASAAAAAGQYGSGPGQQGPYGPGQSGSGQQGPGQQGPYASAAAAAGPGQQGPYGPGSSAAAAAGQYGYGPGQQGPYGPGASGQNGPGSGQYGPGQQGPGQSAAAAAGPGQQGPYGPGASAAAAAGQYGPGQQGPGQYGPGSSGPGQQGPYGPGSSAAAAAGQYGPGQQGPYGPGQSAAAAAGQYQQGPGQQGPYGPGASGPGQQGPYGPGASAAAAAGPGQYGPGQQGPSASAAAAAGQYGSGPGQYGPYGPGQSGPGSGQQGQGPYGPGASAAAAAGQYGPGQQGPYGPGQSAAAAAGPGSGQYGPGASGQNGPGSGQYGPGQQGPGQSAAAAAGQYQQGPGQQGPYGPGASAAAAAGQYGSGPGQQGPYGPGQSGSGQQGPGQQGPYASAAAAAGPGSGQQGPGASGQQGPYGPGASAAAAAGQNGPGSGQQGPGQSGQYGPGQQGPGQQGPGSSAAAAAGPGQYGPGQQGPSASAAAAAGPGSGQQGPGASGQYGPGQQGPGQQGPGSSAAAAAGQYGSGPGQQGPYGSAAAAAGPGSGQYGQGPYGPGASGPGQYGPGQQGPSASAAAAAGSGQQGPGQYGPYASAAAAAGQYGSGPGQQGPYGPGQSGSGQQGPGQQGPYASAAAAAGPGQQGPYGPGSSAAAAAGQYGYGPGQQGPYGPGASGQNGPGSGQYGPGQQGPGQSAAAAAGPGQQGPYGPGASAAAAAGQYGPGQQGPGQYGPGSSGPGQQGPYGPGSSAAAAAGQYGPGQQGPYGPGQSAAAAAGQYQQGPGQQGPYGPGASGPGQQGPYGPGASAAAAAGPGQYGPGQQGPSASAAAAAGQYGSGPGQYGPYGPGQSGPGSGQQGQGPYGPGASAAAAAGQYGPGQQGPYGPGQSAAAAAGPGSGQYGPGASGQNGPGSGQYGPGQQGPGQSAAAAAGQYQQGPGQQGPYGPGASAAAAAGQYGSGPGQQGPYGPGQSGSGQQGPGQQGPYASAAAAAGPGSGQQGPGASGQQGPYGPGASAAAAAGQNGPGSGQQGPGQSGQYGPGQQGPGQQGPGSSAAAAAGPGQYGPGQQGPSASAAAAAGPGSGQQGPGASGQYGPGQQGPGQQGPGSSAAAAAGQYGSGPGQQGPYGSAAAAAGPGSGQYGQGPYGPGASGPGQYGPGQQGPSASAAAAAGSGQQGPGQYGPYASAAAAAGQYGSGPGQQGPYGPGQSGSGQQGPGQQGPYASAAAAAGPGQQGPYGPGSSAAAAAGQYGYGPGQQGPYGPGASGQNGPGSGQYGPGQQGPGQSAAAAAGPGQQGPYGPGASAAAAAGQYGPGQQGPGQYGPGSSGPGQQGPYGPGSSAAAAAGQYGPGQQGPYGPGQSAAAAAGQYQQGPGQQGPYGPGASGPGQQGPYGPGASAAAAAGPGQYGPGQQGPSASAAAAAGQYGSGPGQYGPYGPGQSGPGSGQQGQGPYGPGASAAAAAGQYGPGQQGPYGPGQSAAAAAGPGSGQYGPGASGQNGPGSGQYGPGQQGPGQSAAAAAGQYQQGPGQQGPYGPGASAAAAAGQYGSGPGQQGPYGPGQSGSGQQGPGQQGPYASAAAAAGPGSGQQGPGASGQQGPYGPGASAAAAAGQNGPGSGQQGPGQSGQYGPGQQGPGQQGPGSSAAAAAGPGQYGPGQQGPSASAAAAAGPGSGQQGPGASGQYGPGQQGPGQQGPGSSAAAAAGQYGSGPGQQGPYGSAAAAAGPGSGQYGQGPYGPGASGPGQYGPGQQGPSASAAAAAGSGQQGPGQYGPYASAAAAAGQYGSGPGQQGPYGPGQSGSGQQGPGQQGPYASAAAAAGPGQQGPYGPGSSAAAAAGQYGYGPGQQGPYGPGASGQNGPGSGQYGPGQQGPGQSAAAAAGPGQQGPYGPGASAAAAAGQYGPGQQGPGQYGPGSSGPGQQGPYGPGSSAAAAAGQYGPGQQGPYGPGQSAAAAAGQYQQGPGQQGPYGPGASGPGQQGPYGPGASAAAAAGPGQYGPGQQGPSASAAAAAGQYGSGPGQYGPYGPGQSGPGSGQQGQGPYGPGASAAAAAGQYGPGQQGPYGPGQSAAAAAGPGSGQYGPGASGQNGPGSGQYGPGQQGPGQSAAAAAGQYQQGPGQQGPYGPGASAAAAAGQYGSGPGQQGPYGPGQSGSGQQGPGQQGPYASAAAAAGPGSGQQGSSVDKLAAALEHHHHHH

SEQ ID NO: 10 - protein, 597 aa, Artificial Sequence
  Met-PRT313
MGPGGQGPYGPGASAAAAAGGNGPGSGQQGPGGSAAAAAGGYGPGGQGPGQQGPGSSAAAAAGPGGYGPGGQGPSASAAAAAGPGSGQQGPGASAAAAAGGYGPGGQGPGQQGPGSSAAAAAGGYGSGPGQQGPYGSAAAAAGPGSGGYGQGPYGPGASAAAAAGPGGYGPGGQGPSASAAAAAGSGQQGPGGYGPYASAAAAAGGYGSGPGQQGPYGPGGSAAAAAGSGQQGPGQQGPYASAAAAAGPGGQGPYGPGSSAAAAAGGYGYGPGGQGPYGPGASAAAAAGGNGPGSGGYGPGQQGPGGSAAAAAGPGGQGPYGPGASAAAAAGGYGPGGQGPGGYGPGSSAAAAAGPGGQGPYGPGSSAAAAAGGYGPGQQGPYGPGGSAAAAAGGYQQGPGGQGPYGPGASAAAAAGPGGQGPYGPGASAAAAAGPGGYGPGGQGPSASAAAAAGGYGSGPGGYGPYGPGGSAAAAAGPGSGQQGQGPYGPGASAAAAAGGYGPGQQGPYGPGGSAAAAAGPGSGGYGPGASAAAAAGGNGPGSGGYGPGQQGPGGSAAAAAGGYQQGPGGQGPYGPGASAAAAAGPGSGQQGPGAS

SEQ ID NO: 11 - protein, 12 aa, Artificial Sequence
  HisTag
MHHHHHHSSGSS

SEQ ID NO: 12 - protein, 608 aa, Artificial Sequence
  PRT380
MHHHHHHSSGSSGPGQQGPYGPGASAAAAAGQNGPGSGQQGPGQSAAAAAGQYGPGQQGPGQQGPGSSAAAAAGPGQYGPGQQGPSASAAAAAGPGSGQQGPGASAAAAAGQYGPGQQGPGQQGPGSSAAAAAGQYGSGPGQQGPYGSAAAAAGPGSGQYGQGPYGPGASAAAAAGPGQYGPGQQGPSASAAAAAGSGQQGPGQYGPYASAAAAAGQYGSGPGQQGPYGPGQSAAAAAGSGQQGPGQQGPYASAAAAAGPGQQGPYGPGSSAAAAAGQYGYGPGQQGPYGPGASAAAAAGQNGPGSGQYGPGQQGPGQSAAAAAGPGQQGPYGPGASAAAAAGQYGPGQQGPGQYGPGSSAAAAAGPGQQGPYGPGSSAAAAAGQYGPGQQGPYGPGQSAAAAAGQYQQGPGQQGPYGPGASAAAAAGPGQQGPYGPGASAAAAAGPGQYGPGQQGPSASAAAAAGQYGSGPGQYGPYGPGQSAAAAAGPGSGQQGQGPYGPGASAAAAAGQYGPGQQGPYGPGQSAAAAAGPGSGQYGPGASAAAAAGQNGPGSGQYGPGQQGPGQSAAAAAGQYQQGPGQQGPYGPGASAAAAAGPGSGQQGPGAS

SEQ ID NO: 13 - protein, 601 aa, Artificial Sequence
  PRT410
MHHHHHHSSGSSGPGQQGPYGPGASAAAAAGQNGPGSGQQGPGQSGQYGPGQQGPGQQGPGSSAAAAAGPGQYGPGQQGPSASAAAAAGPGSGQQGPGASGQYGPGQQGPGQQGPGSSAAAAAGQYGSGPGQQGPYGSAAAAAGPGSGQYGQGPYGPGASGPGQYGPGQQGPSASAAAAAGSGQQGPGQYGPYASAAAAAGQYGSGPGQQGPYGPGQSGSGQQGPGQQGPYASAAAAAGPGQQGPYGPGSSAAAAAGQYGYGPGQQGPYGPGASGQNGPGSGQYGPGQQGPGQSAAAAAGPGQQGPYGPGASAAAAAGQYGPGQQGPGQYGPGSSGPGQQGPYGPGSSAAAAAGQYGPGQQGPYGPGQSAAAAAGQYQQGPGQQGPYGPGASGPGQQGPYGPGASAAAAAGPGQYGPGQQGPSASAAAAAGQYGSGPGQYGPYGPGQSGPGSGQQGQGPYGPGASAAAAAGQYGPGQQGPYGPGQSAAAAAGPGSGQYGPGASGQNGPGSGQYGPGQQGPGQSAAAAAGQYQQGPGQQGPYGPGASAAAAAGQYGSGPGQQGPYGPGQSGSGQQGPGQQGPYASAAAAAGPGSGQQGPGAS

SEQ ID NO: 14 - protein, 576 aa, Artificial Sequence
  PRT525
MHHHHHHSSGSSGPGQQGPYGPGASAAAAAAAGSNGPGSGQQGPGQSGQYGPGQQGPGQQGPGSSAAAAAAAGPGQYGPGQQGPSASAAAAAAAGPGSGQQGPGASGQYGPGQQGPGQQGPGSSAAAAAAAGSYGSGPGQQGPYGSAAAAAAAGPGSGQYGQGPYGPGASGPGQYGPGQQGPSASAAAAAAAGSGQQGPGQYGPYASAAAAAAAGSYGSGPGQQGPYGPGQSGSGQQGPGQQGPYASAAAAAAAGPGQQGPYGPGSSAAAAAAAGSYGYGPGQQGPYGPGASGQNGPGSGQYGPGQQGPGPSAAAAAAAGPGQQGPYGPGASAAAAAAAGSYGPGQQGPGQYGPGSSGPGQQGPYGPGSSAAAAAAAGSYGPGQQGPYGPGPSAAAAAAAGSYQQGPGQQGPYGPGASGPGQQGPYGPGASAAAAAAAGPGQYGPGQQGPSASAAAAAAAGSYGSGPGQYGPYGPGQSGPGSGQQGQGPYGPGASAAAAAAAGSYGPGQQGPYGPGPSAAAAAAAGPGSGQYGPGASGQNGPGSGQYGPGQQGPGPSAAAAAAAGPGSGQQGPGAS

SEQ ID NO: 15 - protein, 2375 aa, Artificial Sequence
  PRT799
MHHHHHHSSGSSGPGQQGPYGPGASAAAAAGQNGPGSGQQGPGQSGQYGPGQQGPGQQGPGSSAAAAAGPGQYGPGQQGPSASAAAAAGPGSGQQGPGASGQYGPGQQGPGQQGPGSSAAAAAGQYGSGPGQQGPYGSAAAAAGPGSGQYGQGPYGPGASGPGQYGPGQQGPSASAAAAAGSGQQGPGQYGPYASAAAAAGQYGSGPGQQGPYGPGQSGSGQQGPGQQGPYASAAAAAGPGQQGPYGPGSSAAAAAGQYGYGPGQQGPYGPGASGQNGPGSGQYGPGQQGPGQSAAAAAGPGQQGPYGPGASAAAAAGQYGPGQQGPGQYGPGSSGPGQQGPYGPGSSAAAAAGQYGPGQQGPYGPGQSAAAAAGQYQQGPGQQGPYGPGASGPGQQGPYGPGASAAAAAGPGQYGPGQQGPSASAAAAAGQYGSGPGQYGPYGPGQSGPGSGQQGQGPYGPGASAAAAAGQYGPGQQGPYGPGQSAAAAAGPGSGQYGPGASGQNGPGSGQYGPGQQGPGQSAAAAAGQYQQGPGQQGPYGPGASAAAAAGQYGSGPGQQGPYGPGQSGSGQQGPGQQGPYASAAAAAGPGSGQQGPGASGQQGPYGPGASAAAAAGQNGPGSGQQGPGQSGQYGPGQQGPGQQGPGSSAAAAAGPGQYGPGQQGPSASAAAAAGPGSGQQGPGASGQYGPGQQGPGQQGPGSSAAAAAGQYGSGPGQQGPYGSAAAAAGPGSGQYGQGPYGPGASGPGQYGPGQQGPSASAAAAAGSGQQGPGQYGPYASAAAAAGQYGSGPGQQGPYGPGQSGSGQQGPGQQGPYASAAAAAGPGQQGPYGPGSSAAAAAGQYGYGPGQQGPYGPGASGQNGPGSGQYGPGQQGPGQSAAAAAGPGQQGPYGPGASAAAAAGQYGPGQQGPGQYGPGSSGPGQQGPYGPGSSAAAAAGQYGPGQQGPYGPGQSAAAAAGQYQQGPGQQGPYGPGASGPGQQGPYGPGASAAAAAGPGQYGPGQQGPSASAAAAAGQYGSGPGQYGPYGPGQSGPGSGQQGQGPYGPGASAAAAAGQYGPGQQGPYGPGQSAAAAAGPGSGQYGPGASGQNGPGSGQYGPGQQGPGQSAAAAAGQYQQGPGQQGPYGPGASAAAAAGQYGSGPGQQGPYGPGQSGSGQQGPGQQGPYASAAAAAGPGSGQQGPGASGQQGPYGPGASAAAAAGQNGPGSGQQGPGQSGQYGPGQQGPGQQGPGSSAAAAAGPGQYGPGQQGPSASAAAAAGPGSGQQGPGASGQYGPGQQGPGQQGPGSSAAAAAGQYGSGPGQQGPYGSAAAAAGPGSGQYGQGPYGPGASGPGQYGPGQQGPSASAAAAAGSGQQGPGQYGPYASAAAAAGQYGSGPGQQGPYGPGQSGSGQQGPGQQGPYASAAAAAGPGQQGPYGPGSSAAAAAGQYGYGPGQQGPYGPGASGQNGPGSGQYGPGQQGPGQSAAAAAGPGQQGPYGPGASAAAAAGQYGPGQQGPGQYGPGSSGPGQQGPYGPGSSAAAAAGQYGPGQQGPYGPGQSAAAAAGQYQQGPGQQGPYGPGASGPGQQGPYGPGASAAAAAGPGQYGPGQQGPSASAAAAAGQYGSGPGQYGPYGPGQSGPGSGQQGQGPYGPGASAAAAAGQYGPGQQGPYGPGQSAAAAAGPGSGQYGPGASGQNGPGSGQYGPGQQGPGQSAAAAAGQYQQGPGQQGPYGPGASAAAAAGQYGSGPGQQGPYGPGQSGSGQQGPGQQGPYASAAAAAGPGSGQQGPGASGQQGPYGPGASAAAAAGQNGPGSGQQGPGQSGQYGPGQQGPGQQGPGSSAAAAAGPGQYGPGQQGPSASAAAAAGPGSGQQGPGASGQYGPGQQGPGQQGPGSSAAAAAGQYGSGPGQQGPYGSAAAAAGPGSGQYGQGPYGPGASGPGQYGPGQQGPSASAAAAAGSGQQGPGQYGPYASAAAAAGQYGSGPGQQGPYGPGQSGSGQQGPGQQGPYASAAAAAGPGQQGPYGPGSSAAAAAGQYGYGPGQQGPYGPGASGQNGPGSGQYGPGQQGPGQSAAAAAGPGQQGPYGPGASAAAAAGQYGPGQQGPGQYGPGSSGPGQQGPYGPGSSAAAAAGQYGPGQQGPYGPGQSAAAAAGQYQQGPGQQGPYGPGASGPGQQGPYGPGASAAAAAGPGQYGPGQQGPSASAAAAAGQYGSGPGQYGPYGPGQSGPGSGQQGQGPYGPGASAAAAAGQYGPGQQGPYGPGQSAAAAAGPGSGQYGPGASGQNGPGSGQYGPGQQGPGQSAAAAAGQYQQGPGQQGPYGPGASAAAAAGQYGSGPGQQGPYGPGQSGSGQQGPGQQGPYASAAAAAGPGSGQQGSSVDKLAAALEHHHHHH

SEQ ID NO: 16 - protein, 608 aa, Artificial Sequence
  PRT313
MHHHHHHSSGSSGPGGQGPYGPGASAAAAAGGNGPGSGQQGPGGSAAAAAGGYGPGGQGPGQQGPGSSAAAAAGPGGYGPGGQGPSASAAAAAGPGSGQQGPGASAAAAAGGYGPGGQGPGQQGPGSSAAAAAGGYGSGPGQQGPYGSAAAAAGPGSGGYGQGPYGPGASAAAAAGPGGYGPGGQGPSASAAAAAGSGQQGPGGYGPYASAAAAAGGYGSGPGQQGPYGPGGSAAAAAGSGQQGPGQQGPYASAAAAAGPGGQGPYGPGSSAAAAAGGYGYGPGGQGPYGPGASAAAAAGGNGPGSGGYGPGQQGPGGSAAAAAGPGGQGPYGPGASAAAAAGGYGPGGQGPGGYGPGSSAAAAAGPGGQGPYGPGSSAAAAAGGYGPGQQGPYGPGGSAAAAAGGYQQGPGGQGPYGPGASAAAAAGPGGQGPYGPGASAAAAAGPGGYGPGGQGPSASAAAAAGGYGSGPGGYGPYGPGGSAAAAAGPGSGQQGQGPYGPGASAAAAAGGYGPGQQGPYGPGGSAAAAAGPGSGGYGPGASAAAAAGGNGPGSGGYGPGQQGPGGSAAAAAGGYQQGPGGQGPYGPGASAAAAAGPGSGQQGPGAS

SEQ ID NO: 17 - protein, 590 aa, Artificial Sequence
  Met-PRT399
MGPGGQGPYGPGASAAAAAGGNGPGSGQQGPGGSGGYGPGGQGPGQQGPGSSAAAAAGPGGYGPGGQGPSASAAAAAGPGSGQQGPGASGGYGPGGQGPGQQGPGSSAAAAAGGYGSGPGQQGPYGSAAAAAGPGSGGYGQGPYGPGASGPGGYGPGGQGPSASAAAAAGSGQQGPGGYGPYASAAAAAGGYGSGPGQQGPYGPGGSGSGQQGPGQQGPYASAAAAAGPGGQGPYGPGSSAAAAAGGYGYGPGGQGPYGPGASGGNGPGSGGYGPGQQGPGGSAAAAAGPGGQGPYGPGASAAAAAGGYGPGGQGPGGYGPGSSGPGGQGPYGPGSSAAAAAGGYGPGQQGPYGPGGSAAAAAGGYQQGPGGQGPYGPGASGPGGQGPYGPGASAAAAAGPGGYGPGGQGPSASAAAAAGGYGSGPGGYGPYGPGGSGPGSGQQGQGPYGPGASAAAAAGGYGPGQQGPYGPGGSAAAAAGPGSGGYGPGASGGNGPGSGGYGPGQQGPGGSAAAAAGGYQQGPGGQGPYGPGASAAAAAGGYGSGPGQQGPYGPGGSGSGQQGPGQQGPYASAAAAAGPGSGQQGPGAS

SEQ ID NO: 18 - protein, 601 aa, Artificial Sequence
  PRT399
MHHHHHHSSGSSGPGGQGPYGPGASAAAAAGGNGPGSGQQGPGGSGGYGPGGQGPGQQGPGSSAAAAAGPGGYGPGGQGPSASAAAAAGPGSGQQGPGASGGYGPGGQGPGQQGPGSSAAAAAGGYGSGPGQQGPYGSAAAAAGPGSGGYGQGPYGPGASGPGGYGPGGQGPSASAAAAAGSGQQGPGGYGPYASAAAAAGGYGSGPGQQGPYGPGGSGSGQQGPGQQGPYASAAAAAGPGGQGPYGPGSSAAAAAGGYGYGPGGQGPYGPGASGGNGPGSGGYGPGQQGPGGSAAAAAGPGGQGPYGPGASAAAAAGGYGPGGQGPGGYGPGSSGPGGQGPYGPGSSAAAAAGGYGPGQQGPYGPGGSAAAAAGGYQQGPGGQGPYGPGASGPGGQGPYGPGASAAAAAGPGGYGPGGQGPSASAAAAAGGYGSGPGGYGPYGPGGSGPGSGQQGQGPYGPGASAAAAAGGYGPGQQGPYGPGGSAAAAAGPGSGGYGPGASGGNGPGSGGYGPGQQGPGGSAAAAAGGYQQGPGGQGPYGPGASAAAAAGGYGSGPGQQGPYGPGGSGSGQQGPGQQGPYASAAAAAGPGSGQQGPGAS

SEQ ID NO: 19 - protein, 612 aa, Artificial Sequence
  Met-PRT720
MGPGQQGPYGPGASAAAAAGQNGPGSGQQGPGQSGQYGPGQQGPGQQGPGSSAAAAAGPGQYVLIGPGQQVLIGPSASAAAAAGPGSGQQGPGASGQYGPGQQGPGQQGPGSSAAAAAGSYGSVLIGPGQQVLIGPYGSAAAAAGPGSGQYGQGPYGPGASGPGQYGPGQQGPSASAAAAAGSGQQVLIGPGQYVLIGPYASAAAAAGQYGSGPGQQGPYGPGQSGSGQQGPGQQGPYASAAAAAGPGQQVLIGPYVLIGPGSSAAAAAGQYGYGPGQQGPYGPGASGQNGPGSGQYGPGQQGPGQSAAAAAGPGQQVLIGPYVLIGPGASAAAAAGQYGPGQQGPGQYGPGSSGPGQQGPYGPGSSAAAAAGSYGPGQQVLIGPYVLIGPGPSAAAAAGQYQQGPGQQGPYGPGASGPGQQGPYGPGASAAAAAGPGQYVLIGPGQQVLIGPSASAAAAAGQYGSGPGQYGPYGPGQSGPGSGQQGQGPYGPGASAAAAAGSYGPGQQVLIGPYVLIGPGPSAAAAAGPGSGQYGPGASGQNGPGSGQYGPGQQGPGQSAAAAAGQYQQVLIGPGQQGPYVLIGPGASAAAAAGPGSGQQVLIGPGASVLI

SEQ ID NO: 20 - protein, 592 aa, Artificial Sequence
  Met-PRT665
MGPGQQGPYGPGASAAAAAAAGSNGPGSGQQGPGQSGQYGPGQQGPGQQGPGSSAAAAAAAGPGQYVLIGPGQQGPSASAAAAAAAGPGSGQQGPGASGQYGPGQQGPGQQGPGSSAAAAAAAGSYGSVLIGPGQQGPYGSAAAAAAAGPGSGQYGQGPYGPGASGPGQYGPGQQGPSASAAAAAAAGSGQQVLIGPGQYGPYASAAAAAAAGSYGSGPGQQGPYGPGQSGSGQQGPGQQGPYASAAAAAAAGPGQQVLIGPYGPGSSAAAAAAAGSYGYGPGQQGPYGPGASGQNGPGSGQYGPGQQGPGPSAAAAAAAGPGQQVLIGPYGPGASAAAAAAAGSYGPGQQGPGQYGPGSSGPGQQGPYGPGSSAAAAAAAGSYGPGQQVLIGPYGPGPSAAAAAAAGSYQQGPGQQGPYGPGASGPGQQGPYGPGASAAAAAAAGPGQYVLIGPGQQGPSASAAAAAAAGSYGSGPGQYGPYGPGQSGPGSGQQGQGPYGPGASAAAAAAAGSYGPGQQVLIGPYGPGPSAAAAAAAGPGSGQYGPGASGQNGPGSGQYGPGQQGPGPSAAAAAAAGPGSGQQGPGASVLI

SEQ ID NO: 21 - protein, 619 aa, Artificial Sequence
  Met-PRT666
MGPGQQGPYGPGASAAAAAAAGSNGPGSGQQGPGQSGQYGPGQQGPGQQGPGSSAAAAAAAGPGQYVLIGPGQQVLIGPSASAAAAAAAGPGSGQQGPGASGQYGPGQQGPGQQGPGSSAAAAAAAGSYGSVLIGPGQQVLIGPYGSAAAAAAAGPGSGQYGQGPYGPGASGPGQYGPGQQGPSASAAAAAAAGSGQQVLIGPGQYVLIGPYASAAAAAAAGSYGSGPGQQGPYGPGQSGSGQQGPGQQGPYASAAAAAAAGPGQQVLIGPYVLIGPGSSAAAAAAAGSYGYGPGQQGPYGPGASGQNGPGSGQYGPGQQGPGPSAAAAAAAGPGQQVLIGPYVLIGPGASAAAAAAAGSYGPGQQGPGQYGPGSSGPGQQGPYGPGSSAAAAAAAGSYGPGQQVLIGPYVLIGPGPSAAAAAAAGSYQQGPGQQGPYGPGASGPGQQGPYGPGASAAAAAAAGPGQYVLIGPGQQVLIGPSASAAAAAAAGSYGSGPGQYGPYGPGQSGPGSGQQGQGPYGPGASAAAAAAAGSYGPGQQVLIGPYVLIGPGPSAAAAAAAGPGSGQYGPGASGQNGPGSGQYGPGQQGPGPSAAAAAAAGPGSGQQVLIGPGASVLI

SEQ ID NO: 22 - protein, 623 aa, Artificial Sequence
  PRT720
MHHHHHHSSGSSGPGQQGPYGPGASAAAAAGQNGPGSGQQGPGQSGQYGPGQQGPGQQGPGSSAAAAAGPGQYVLIGPGQQVLIGPSASAAAAAGPGSGQQGPGASGQYGPGQQGPGQQGPGSSAAAAAGSYGSVLIGPGQQVLIGPYGSAAAAAGPGSGQYGQGPYGPGASGPGQYGPGQQGPSASAAAAAGSGQQVLIGPGQYVLIGPYASAAAAAGQYGSGPGQQGPYGPGQSGSGQQGPGQQGPYASAAAAAGPGQQVLIGPYVLIGPGSSAAAAAGQYGYGPGQQGPYGPGASGQNGPGSGQYGPGQQGPGQSAAAAAGPGQQVLIGPYVLIGPGASAAAAAGQYGPGQQGPGQYGPGSSGPGQQGPYGPGSSAAAAAGSYGPGQQVLIGPYVLIGPGPSAAAAAGQYQQGPGQQGPYGPGASGPGQQGPYGPGASAAAAAGPGQYVLIGPGQQVLIGPSASAAAAAGQYGSGPGQYGPYGPGQSGPGSGQQGQGPYGPGASAAAAAGSYGPGQQVLIGPYVLIGPGPSAAAAAGPGSGQYGPGASGQNGPGSGQYGPGQQGPGQSAAAAAGQYQQVLIGPGQQGPYVLIGPGASAAAAAGPGSGQQVLIGPGASVLI

SEQ ID NO: 23 - protein, 603 aa, Artificial Sequence
  PRT665
MHHHHHHSSGSSGPGQQGPYGPGASAAAAAAAGSNGPGSGQQGPGQSGQYGPGQQGPGQQGPGSSAAAAAAAGPGQYVLIGPGQQGPSASAAAAAAAGPGSGQQGPGASGQYGPGQQGPGQQGPGSSAAAAAAAGSYGSVLIGPGQQGPYGSAAAAAAAGPGSGQYGQGPYGPGASGPGQYGPGQQGPSASAAAAAAAGSGQQVLIGPGQYGPYASAAAAAAAGSYGSGPGQQGPYGPGQSGSGQQGPGQQGPYASAAAAAAAGPGQQVLIGPYGPGSSAAAAAAAGSYGYGPGQQGPYGPGASGQNGPGSGQYGPGQQGPGPSAAAAAAAGPGQQVLIGPYGPGASAAAAAAAGSYGPGQQGPGQYGPGSSGPGQQGPYGPGSSAAAAAAAGSYGPGQQVLIGPYGPGPSAAAAAAAGSYQQGPGQQGPYGPGASGPGQQGPYGPGASAAAAAAAGPGQYVLIGPGQQGPSASAAAAAAAGSYGSGPGQYGPYGPGQSGPGSGQQGQGPYGPGASAAAAAAAGSYGPGQQVLIGPYGPGPSAAAAAAAGPGSGQYGPGASGQNGPGSGQYGPGQQGPGPSAAAAAAAGPGSGQQGPGASVLI

SEQ ID NO: 24 - protein, 630 aa, Artificial Sequence
  PRT666
MHHHHHHSSGSSGPGQQGPYGPGASAAAAAAAGSNGPGSGQQGPGQSGQYGPGQQGPGQQGPGSSAAAAAAAGPGQYVLIGPGQQVLIGPSASAAAAAAAGPGSGQQGPGASGQYGPGQQGPGQQGPGSSAAAAAAAGSYGSVLIGPGQQVLIGPYGSAAAAAAAGPGSGQYGQGPYGPGASGPGQYGPGQQGPSASAAAAAAAGSGQQVLIGPGQYVLIGPYASAAAAAAAGSYGSGPGQQGPYGPGQSGSGQQGPGQQGPYASAAAAAAAGPGQQVLIGPYVLIGPGSSAAAAAAAGSYGYGPGQQGPYGPGASGQNGPGSGQYGPGQQGPGPSAAAAAAAGPGQQVLIGPYVLIGPGASAAAAAAAGSYGPGQQGPGQYGPGSSGPGQQGPYGPGSSAAAAAAAGSYGPGQQVLIGPYVLIGPGPSAAAAAAAGSYQQGPGQQGPYGPGASGPGQQGPYGPGASAAAAAAAGPGQYVLIGPGQQVLIGPSASAAAAAAAGSYGSGPGQYGPYGPGQSGPGSGQQGQGPYGPGASAAAAAAAGSYGPGQQVLIGPYVLIGPGPSAAAAAAAGPGSGQYGPGASGQNGPGSGQYGPGQQGPGPSAAAAAAAGPGSGQQVLIGPGASVLI

SEQ ID NO: 25 - protein, 593 aa, Artificial Sequence
  Met-PRT888
MGSSGPGVLGPYGPGASAAAAAGQNGPGSGVLGPGQSGQYGPGVLGPGVLGPGSSAAAAAGPGQYGPGVLGPSASAAAAAGPGSGVLGPGASGQYGPGVLGPGVLGPGSSAAAAAGQYGSGPGVLGPYGSAAAAAGPGSGQYGQGPYGPGASGPGQYGPGVLGPSASAAAAAGSGVLGPGQYGPYASAAAAAGQYGSGPGVLGPYGPGQSGSGVLGPGVLGPYASAAAAAGPGVLGPYGPGSSAAAAAGQYGYGPGVLGPYGPGASGQNGPGSGQYGPGVLGPGQSAAAAAGPGVLGPYGPGASAAAAAGQYGPGVLGPGQYGPGSSGPGVLGPYGPGSSAAAAAGQYGPGVLGPYGPGQSAAAAAGQYVLGPGVLGPYGPGASGPGVLGPYGPGASAAAAAGPGQYGPGVLGPSASAAAAAGQYGSGPGQYGPYGPGQSGPGSGVLGQGPYGPGASAAAAAGQYGPGVLGPYGPGQSAAAAAGPGSGQYGPGASGQNGPGSGQYGPGVLGPGQSAAAAAGQYVLGPGVLGPYGPGASAAAAAGQYGSGPGVLGPYGPGQSGSGVLGPGVLGPYASAAAAAGPGSGVLGPGAS

SEQ ID NO: 26 - protein, 590 aa, Artificial Sequence
  Met-PRT965
MGPGTSGPYGPGASAAAAAGANGPGSGTSGPGASGAYGPGTSGPGTSGPGSSAAAAAGPGAYGPGTSGPSASAAAAAGPGSGTSGPGASGAYGPGTSGPGTSGPGSSAAAAAGAYGSGPGTSGPYGSAAAAAGPGSGAYGAGPYGPGASGPGAYGPGTSGPSASAAAAAGSGTSGPGAYGPYASAAAAAGAYGSGPGTSGPYGPGASGSGTSGPGTSGPYASAAAAAGPGTSGPYGPGSSAAAAAGAYGYGPGTSGPYGPGASGANGPGSGAYGPGTSGPGASAAAAAGPGTSGPYGPGASAAAAAGAYGPGTSGPGAYGPGSSGPGTSGPYGPGSSAAAAAGAYGPGTSGPYGPGASAAAAAGAYTSGPGTSGPYGPGASGPGTSGPYGPGASAAAAAGPGAYGPGTSGPSASAAAAAGAYGSGPGAYGPYGPGASGPGSGTSGAGPYGPGASAAAAAGAYGPGTSGPYGPGASAAAAAGPGSGAYGPGASGANGPGSGAYGPGTSGPGASAAAAAGAYTSGPGTSGPYGPGASAAAAAGAYGSGPGTSGPYGPGASGSGTSGPGTSGPYASAAAAAGPGSGTSGPGAS

SEQ ID NO: 27 - protein, 593 aa, Artificial Sequence
  Met-PRT889
MGSSGPGVLGPYGPGASAAAAAGINGPGSGVLGPGISGIYGPGVLGPGVLGPGSSAAAAAGPGIYGPGVLGPSASAAAAAGPGSGVLGPGASGIYGPGVLGPGVLGPGSSAAAAAGIYGSGPGVLGPYGSAAAAAGPGSGIYGIGPYGPGASGPGIYGPGVLGPSASAAAAAGSGVLGPGIYGPYASAAAAAGIYGSGPGVLGPYGPGISGSGVLGPGVLGPYASAAAAAGPGVLGPYGPGSSAAAAAGIYGYGPGVLGPYGPGASGINGPGSGIYGPGVLGPGISAAAAAGPGVLGPYGPGASAAAAAGIYGPGVLGPGIYGPGSSGPGVLGPYGPGSSAAAAAGIYGPGVLGPYGPGISAAAAAGIYVLGPGVLGPYGPGASGPGVLGPYGPGASAAAAAGPGIYGPGVLGPSASAAAAAGIYGSGPGIYGPYGPGISGPGSGVLGIGPYGPGASAAAAAGIYGPGVLGPYGPGISAAAAAGPGSGIYGPGASGINGPGSGIYGPGVLGPGISAAAAAGIYVLGPGVLGPYGPGASAAAAAGIYGSGPGVLGPYGPGISGSGVLGPGVLGPYASAAAAAGPGSGVLGPGAS

SEQ ID NO: 28 - protein, 590 aa, Artificial Sequence
  Met-PRT916
MGPGVIGPYGPGASAAAAAGLNGPGSGVIGPGLSGLYGPGVIGPGVIGPGSSAAAAAGPGLYGPGVIGPSASAAAAAGPGSGVIGPGASGLYGPGVIGPGVIGPGSSAAAAAGLYGSGPGVIGPYGSAAAAAGPGSGLYGLGPYGPGASGPGLYGPGVIGPSASAAAAAGSGVIGPGLYGPYASAAAAAGLYGSGPGVIGPYGPGLSGSGVIGPGVIGPYASAAAAAGPGVIGPYGPGSSAAAAAGLYGYGPGVIGPYGPGASGLNGPGSGLYGPGVIGPGLSAAAAAGPGVIGPYGPGASAAAAAGLYGPGVIGPGLYGPGSSGPGVIGPYGPGSSAAAAAGLYGPGVIGPYGPGLSAAAAAGLYVIGPGVIGPYGPGASGPGVIGPYGPGASAAAAAGPGLYGPGVIGPSASAAAAAGLYGSGPGLYGPYGPGLSGPGSGVIGLGPYGPGASAAAAAGLYGPGVIGPYGPGLSAAAAAGPGSGLYGPGASGLNGPGSGLYGPGVIGPGLSAAAAAGLYVIGPGVIGPYGPGASAAAAAGLYGSGPGVIGPYGPGLSGSGVIGPGVIGPYASAAAAAGPGSGVIGPGAS

SEQ ID NO: 29 - protein, 590 aa, Artificial Sequence
  Met-PRT918
MGPGVFGPYGPGASAAAAAGINGPGSGVFGPGISGIYGPGVFGPGVFGPGSSAAAAAGPGIYGPGVFGPSASAAAAAGPGSGVFGPGASGIYGPGVFGPGVFGPGSSAAAAAGIYGSGPGVFGPYGSAAAAAGPGSGIYGIGPYGPGASGPGIYGPGVFGPSASAAAAAGSGVFGPGIYGPYASAAAAAGIYGSGPGVFGPYGPGISGSGVFGPGVFGPYASAAAAAGPGVFGPYGPGSSAAAAAGIYGYGPGVFGPYGPGASGINGPGSGIYGPGVFGPGISAAAAAGPGVFGPYGPGASAAAAAGIYGPGVFGPGIYGPGSSGPGVFGPYGPGSSAAAAAGIYGPGVFGPYGPGISAAAAAGIYVFGPGVFGPYGPGASGPGVFGPYGPGASAAAAAGPGIYGPGVFGPSASAAAAAGIYGSGPGIYGPYGPGISGPGSGVFGIGPYGPGASAAAAAGIYGPGVFGPYGPGISAAAAAGPGSGIYGPGASGINGPGSGIYGPGVFGPGISAAAAAGIYVFGPGVFGPYGPGASAAAAAGIYGSGPGVFGPYGPGISGSGVFGPGVFGPYASAAAAAGPGSGVFGPGAS

SEQ ID NO: 30 - protein, 565 aa, Artificial Sequence
  Met-PRT699
MGPGVLGPYGPGASAAAAAAAGSNGPGSGVLGPGQSGQYGPGVLGPGVLGPGSSAAAAAAAGPGQYGPGVLGPSASAAAAAAAGPGSGVLGPGASGQYGPGVLGPGVLGPGSSAAAAAAAGSYGSGPGVLGPYGSAAAAAAAGPGSGQYGQGPYGPGASGPGQYGPGVLGPSASAAAAAAAGSGVLGPGQYGPYASAAAAAAAGSYGSGPGVLGPYGPGQSGSGVLGPGVLGPYASAAAAAAAGPGVLGPYGPGSSAAAAAAAGSYGYGPGVLGPYGPGASGQNGPGSGQYGPGVLGPGPSAAAAAAAGPGVLGPYGPGASAAAAAAAGSYGPGVLGPGQYGPGSSGPGVLGPYGPGSSAAAAAAAGSYGPGVLGPYGPGPSAAAAAAAGSYVLGPGVLGPYGPGASGPGVLGPYGPGASAAAAAAAGPGQYGPGVLGPSASAAAAAAAGSYGSGPGQYGPYGPGQSGPGSGVLGQGPYGPGASAAAAAAAGSYGPGVLGPYGPGPSAAAAAAAGPGSGQYGPGASGQNGPGSGQYGPGVLGPGPSAAAAAAAGPGSGVLGPGAS

SEQ ID NO: 31 - protein, 565 aa, Artificial Sequence
  Met-PRT698
MGPGVLGPYGPGASAAAAAAAGSNGPGSGVLGPGISGIYGPGVLGPGVLGPGSSAAAAAAAGPGIYGPGVLGPSASAAAAAAAGPGSGVLGPGASGIYGPGVLGPGVLGPGSSAAAAAAAGSYGSGPGVLGPYGSAAAAAAAGPGSGIYGIGPYGPGASGPGIYGPGVLGPSASAAAAAAAGSGVLGPGIYGPYASAAAAAAAGSYGSGPGVLGPYGPGISGSGVLGPGVLGPYASAAAAAAAGPGVLGPYGPGSSAAAAAAAGSYGYGPGVLGPYGPGASGINGPGSGIYGPGVLGPGPSAAAAAAAGPGVLGPYGPGASAAAAAAAGSYGPGVLGPGIYGPGSSGPGVLGPYGPGSSAAAAAAAGSYGPGVLGPYGPGPSAAAAAAAGSYVLGPGVLGPYGPGASGPGVLGPYGPGASAAAAAAAGPGIYGPGVLGPSASAAAAAAAGSYGSGPGIYGPYGPGISGPGSGVLGIGPYGPGASAAAAAAAGSYGPGVLGPYGPGPSAAAAAAAGPGSGIYGPGASGINGPGSGIYGPGVLGPGPSAAAAAAAGPGSGVLGPGAS

SEQ ID NO: 32 - protein, 1179 aa, Artificial Sequence
  Met-PRT966
MGPGVFGPYGPGASAAAAAGINGPGSGVFGPGISGIYGPGVFGPGVFGPGSSAAAAAGPGIYGPGVFGPSASAAAAAGPGSGVFGPGASGIYGPGVFGPGVFGPGSSAAAAAGIYGSGPGVFGPYGSAAAAAGPGSGIYGIGPYGPGASGPGIYGPGVFGPSASAAAAAGSGVFGPGIYGPYASAAAAAGIYGSGPGVFGPYGPGISGSGVFGPGVFGPYASAAAAAGPGVFGPYGPGSSAAAAAGIYGYGPGVFGPYGPGASGINGPGSGIYGPGVFGPGISAAAAAGPGVFGPYGPGASAAAAAGIYGPGVFGPGIYGPGSSGPGVFGPYGPGSSAAAAAGIYGPGVFGPYGPGISAAAAAGIYVFGPGVFGPYGPGASGPGVFGPYGPGASAAAAAGPGIYGPGVFGPSASAAAAAGIYGSGPGIYGPYGPGISGPGSGVFGIGPYGPGASAAAAAGIYGPGVFGPYGPGISAAAAAGPGSGIYGPGASGINGPGSGIYGPGVFGPGISAAAAAGIYVFGPGVFGPYGPGASAAAAAGIYGSGPGVFGPYGPGISGSGVFGPGVFGPYASAAAAAGPGSGVFGPGASGPGVFGPYGPGASAAAAAGINGPGSGVFGPGISGIYGPGVFGPGVFGPGSSAAAAAGPGIYGPGVFGPSASAAAAAGPGSGVFGPGASGIYGPGVFGPGVFGPGSSAAAAAGIYGSGPGVFGPYGSAAAAAGPGSGIYGIGPYGPGASGPGIYGPGVFGPSASAAAAAGSGVFGPGIYGPYASAAAAAGIYGSGPGVFGPYGPGISGSGVFGPGVFGPYASAAAAAGPGVFGPYGPGSSAAAAAGIYGYGPGVFGPYGPGASGINGPGSGIYGPGVFGPGISAAAAAGPGVFGPYGPGASAAAAAGIYGPGVFGPGIYGPGSSGPGVFGPYGPGSSAAAAAGIYGPGVFGPYGPGISAAAAAGIYVFGPGVFGPYGPGASGPGVFGPYGPGASAAAAAGPGIYGPGVFGPSASAAAAAGIYGSGPGIYGPYGPGISGPGSGVFGIGPYGPGASAAAAAGIYGPGVFGPYGPGISAAAAAGPGSGIYGPGASGINGPGSGIYGPGVFGPGISAAAAAGIYVFGPGVFGPYGPGASAAAAAGIYGSGPGVFGPYGPGISGSGVFGPGVFGPYASAAAAAGPGSGVFGPGAS

SEQ ID NO: 33 - protein, 601 aa, Artificial Sequence
  PRT888
MHHHHHHSSGSSGPGVLGPYGPGASAAAAAGQNGPGSGVLGPGQSGQYGPGVLGPGVLGPGSSAAAAAGPGQYGPGVLGPSASAAAAAGPGSGVLGPGASGQYGPGVLGPGVLGPGSSAAAAAGQYGSGPGVLGPYGSAAAAAGPGSGQYGQGPYGPGASGPGQYGPGVLGPSASAAAAAGSGVLGPGQYGPYASAAAAAGQYGSGPGVLGPYGPGQSGSGVLGPGVLGPYASAAAAAGPGVLGPYGPGSSAAAAAGQYGYGPGVLGPYGPGASGQNGPGSGQYGPGVLGPGQSAAAAAGPGVLGPYGPGASAAAAAGQYGPGVLGPGQYGPGSSGPGVLGPYGPGSSAAAAAGQYGPGVLGPYGPGQSAAAAAGQYVLGPGVLGPYGPGASGPGVLGPYGPGASAAAAAGPGQYGPGVLGPSASAAAAAGQYGSGPGQYGPYGPGQSGPGSGVLGQGPYGPGASAAAAAGQYGPGVLGPYGPGQSAAAAAGPGSGQYGPGASGQNGPGSGQYGPGVLGPGQSAAAAAGQYVLGPGVLGPYGPGASAAAAAGQYGSGPGVLGPYGPGQSGSGVLGPGVLGPYASAAAAAGPGSGVLGPGAS

SEQ ID NO: 34 - protein, 601 aa, Artificial Sequence
  PRT965
MHHHHHHSSGSSGPGTSGPYGPGASAAAAAGANGPGSGTSGPGASGAYGPGTSGPGTSGPGSSAAAAAGPGAYGPGTSGPSASAAAAAGPGSGTSGPGASGAYGPGTSGPGTSGPGSSAAAAAGAYGSGPGTSGPYGSAAAAAGPGSGAYGAGPYGPGASGPGAYGPGTSGPSASAAAAAGSGTSGPGAYGPYASAAAAAGAYGSGPGTSGPYGPGASGSGTSGPGTSGPYASAAAAAGPGTSGPYGPGSSAAAAAGAYGYGPGTSGPYGPGASGANGPGSGAYGPGTSGPGASAAAAAGPGTSGPYGPGASAAAAAGAYGPGTSGPGAYGPGSSGPGTSGPYGPGSSAAAAAGAYGPGTSGPYGPGASAAAAAGAYTSGPGTSGPYGPGASGPGTSGPYGPGASAAAAAGPGAYGPGTSGPSASAAAAAGAYGSGPGAYGPYGPGASGPGSGTSGAGPYGPGASAAAAAGAYGPGTSGPYGPGASAAAAAGPGSGAYGPGASGANGPGSGAYGPGTSGPGASAAAAAGAYTSGPGTSGPYGPGASAAAAAGAYGSGPGTSGPYGPGASGSGTSGPGTSGPYASAAAAAGPGSGTSGPGAS

SEQ ID NO: 35 - protein, 601 aa, Artificial Sequence
  PRT889
MHHHHHHSSGSSGPGVLGPYGPGASAAAAAGINGPGSGVLGPGISGIYGPGVLGPGVLGPGSSAAAAAGPGIYGPGVLGPSASAAAAAGPGSGVLGPGASGIYGPGVLGPGVLGPGSSAAAAAGIYGSGPGVLGPYGSAAAAAGPGSGIYGIGPYGPGASGPGIYGPGVLGPSASAAAAAGSGVLGPGIYGPYASAAAAAGIYGSGPGVLGPYGPGISGSGVLGPGVLGPYASAAAAAGPGVLGPYGPGSSAAAAAGIYGYGPGVLGPYGPGASGINGPGSGIYGPGVLGPGISAAAAAGPGVLGPYGPGASAAAAAGIYGPGVLGPGIYGPGSSGPGVLGPYGPGSSAAAAAGIYGPGVLGPYGPGISAAAAAGIYVLGPGVLGPYGPGASGPGVLGPYGPGASAAAAAGPGIYGPGVLGPSASAAAAAGIYGSGPGIYGPYGPGISGPGSGVLGIGPYGPGASAAAAAGIYGPGVLGPYGPGISAAAAAGPGSGIYGPGASGINGPGSGIYGPGVLGPGISAAAAAGIYVLGPGVLGPYGPGASAAAAAGIYGSGPGVLGPYGPGISGSGVLGPGVLGPYASAAAAAGPGSGVLGPGAS

SEQ ID NO: 36 - protein, 601 aa, Artificial Sequence
  PRT916
MHHHHHHSSGSSGPGVIGPYGPGASAAAAAGLNGPGSGVIGPGLSGLYGPGVIGPGVIGPGSSAAAAAGPGLYGPGVIGPSASAAAAAGPGSGVIGPGASGLYGPGVIGPGVIGPGSSAAAAAGLYGSGPGVIGPYGSAAAAAGPGSGLYGLGPYGPGASGPGLYGPGVIGPSASAAAAAGSGVIGPGLYGPYASAAAAAGLYGSGPGVIGPYGPGLSGSGVIGPGVIGPYASAAAAAGPGVIGPYGPGSSAAAAAGLYGYGPGVIGPYGPGASGLNGPGSGLYGPGVIGPGLSAAAAAGPGVIGPYGPGASAAAAAGLYGPGVIGPGLYGPGSSGPGVIGPYGPGSSAAAAAGLYGPGVIGPYGPGLSAAAAAGLYVIGPGVIGPYGPGASGPGVIGPYGPGASAAAAAGPGLYGPGVIGPSASAAAAAGLYGSGPGLYGPYGPGLSGPGSGVIGLGPYGPGASAAAAAGLYGPGVIGPYGPGLSAAAAAGPGSGLYGPGASGLNGPGSGLYGPGVIGPGLSAAAAAGLYVIGPGVIGPYGPGASAAAAAGLYGSGPGVIGPYGPGLSGSGVIGPGVIGPYASAAAAAGPGSGVIGPGAS

SEQ ID NO: 37 - protein, 601 aa, Artificial Sequence
  PRT918
MHHHHHHSSGSSGPGVFGPYGPGASAAAAAGINGPGSGVFGPGISGIYGPGVFGPGVFGPGSSAAAAAGPGIYGPGVFGPSASAAAAAGPGSGVFGPGASGIYGPGVFGPGVFGPGSSAAAAAGIYGSGPGVFGPYGSAAAAAGPGSGIYGIGPYGPGASGPGIYGPGVFGPSASAAAAAGSGVFGPGIYGPYASAAAAAGIYGSGPGVFGPYGPGISGSGVFGPGVFGPYASAAAAAGPGVFGPYGPGSSAAAAAGIYGYGPGVFGPYGPGASGINGPGSGIYGPGVFGPGISAAAAAGPGVFGPYGPGASAAAAAGIYGPGVFGPGIYGPGSSGPGVFGPYGPGSSAAAAAGIYGPGVFGPYGPGISAAAAAGIYVFGPGVFGPYGPGASGPGVFGPYGPGASAAAAAGPGIYGPGVFGPSASAAAAAGIYGSGPGIYGPYGPGISGPGSGVFGIGPYGPGASAAAAAGIYGPGVFGPYGPGISAAAAAGPGSGIYGPGASGINGPGSGIYGPGVFGPGISAAAAAGIYVFGPGVFGPYGPGASAAAAAGIYGSGPGVFGPYGPGISGSGVFGPGVFGPYASAAAAAGPGSGVFGPGAS

SEQ ID NO: 38 - protein, 576 aa, Artificial Sequence
  PRT699
MHHHHHHSSGSSGPGVLGPYGPGASAAAAAAAGSNGPGSGVLGPGQSGQYGPGVLGPGVLGPGSSAAAAAAAGPGQYGPGVLGPSASAAAAAAAGPGSGVLGPGASGQYGPGVLGPGVLGPGSSAAAAAAAGSYGSGPGVLGPYGSAAAAAAAGPGSGQYGQGPYGPGASGPGQYGPGVLGPSASAAAAAAAGSGVLGPGQYGPYASAAAAAAAGSYGSGPGVLGPYGPGQSGSGVLGPGVLGPYASAAAAAAAGPGVLGPYGPGSSAAAAAAAGSYGYGPGVLGPYGPGASGQNGPGSGQYGPGVLGPGPSAAAAAAAGPGVLGPYGPGASAAAAAAAGSYGPGVLGPGQYGPGSSGPGVLGPYGPGSSAAAAAAAGSYGPGVLGPYGPGPSAAAAAAAGSYVLGPGVLGPYGPGASGPGVLGPYGPGASAAAAAAAGPGQYGPGVLGPSASAAAAAAAGSYGSGPGQYGPYGPGQSGPGSGVLGQGPYGPGASAAAAAAAGSYGPGVLGPYGPGPSAAAAAAAGPGSGQYGPGASGQNGPGSGQYGPGVLGPGPSAAAAAAAGPGSGVLGPGAS

SEQ ID NO: 39 - protein, 576 aa, Artificial Sequence
  PRT698
MHHHHHHSSGSSGPGVLGPYGPGASAAAAAAAGSNGPGSGVLGPGISGIYGPGVLGPGVLGPGSSAAAAAAAGPGIYGPGVLGPSASAAAAAAAGPGSGVLGPGASGIYGPGVLGPGVLGPGSSAAAAAAAGSYGSGPGVLGPYGSAAAAAAAGPGSGIYGIGPYGPGASGPGIYGPGVLGPSASAAAAAAAGSGVLGPGIYGPYASAAAAAAAGSYGSGPGVLGPYGPGISGSGVLGPGVLGPYASAAAAAAAGPGVLGPYGPGSSAAAAAAAGSYGYGPGVLGPYGPGASGINGPGSGIYGPGVLGPGPSAAAAAAAGPGVLGPYGPGASAAAAAAAGSYGPGVLGPGIYGPGSSGPGVLGPYGPGSSAAAAAAAGSYGPGVLGPYGPGPSAAAAAAAGSYVLGPGVLGPYGPGASGPGVLGPYGPGASAAAAAAAGPGIYGPGVLGPSASAAAAAAAGSYGSGPGIYGPYGPGISGPGSGVLGIGPYGPGASAAAAAAAGSYGPGVLGPYGPGPSAAAAAAAGPGSGIYGPGASGINGPGSGIYGPGVLGPGPSAAAAAAAGPGSGVLGPGAS

SEQ ID NO: 40 - protein, 1190 aa, Artificial Sequence
  PRT966
MHHHHHHSSGSSGPGVFGPYGPGASAAAAAGINGPGSGVFGPGISGIYGPGVFGPGVFGPGSSAAAAAGPGIYGPGVFGPSASAAAAAGPGSGVFGPGASGIYGPGVFGPGVFGPGSSAAAAAGIYGSGPGVFGPYGSAAAAAGPGSGIYGIGPYGPGASGPGIYGPGVFGPSASAAAAAGSGVFGPGIYGPYASAAAAAGIYGSGPGVFGPYGPGISGSGVFGPGVFGPYASAAAAAGPGVFGPYGPGSSAAAAAGIYGYGPGVFGPYGPGASGINGPGSGIYGPGVFGPGISAAAAAGPGVFGPYGPGASAAAAAGIYGPGVFGPGIYGPGSSGPGVFGPYGPGSSAAAAAGIYGPGVFGPYGPGISAAAAAGIYVFGPGVFGPYGPGASGPGVFGPYGPGASAAAAAGPGIYGPGVFGPSASAAAAAGIYGSGPGIYGPYGPGISGPGSGVFGIGPYGPGASAAAAAGIYGPGVFGPYGPGISAAAAAGPGSGIYGPGASGINGPGSGIYGPGVFGPGISAAAAAGIYVFGPGVFGPYGPGASAAAAAGIYGSGPGVFGPYGPGISGSGVFGPGVFGPYASAAAAAGPGSGVFGPGASGPGVFGPYGPGASAAAAAGINGPGSGVFGPGISGIYGPGVFGPGVFGPGSSAAAAAGPGIYGPGVFGPSASAAAAAGPGSGVFGPGASGIYGPGVFGPGVFGPGSSAAAAAGIYGSGPGVFGPYGSAAAAAGPGSGIYGIGPYGPGASGPGIYGPGVFGPSASAAAAAGSGVFGPGIYGPYASAAAAAGIYGSGPGVFGPYGPGISGSGVFGPGVFGPYASAAAAAGPGVFGPYGPGSSAAAAAGIYGYGPGVFGPYGPGASGINGPGSGIYGPGVFGPGISAAAAAGPGVFGPYGPGASAAAAAGIYGPGVFGPGIYGPGSSGPGVFGPYGPGSSAAAAAGIYGPGVFGPYGPGISAAAAAGIYVFGPGVFGPYGPGASGPGVFGPYGPGASAAAAAGPGIYGPGVFGPSASAAAAAGIYGSGPGIYGPYGPGISGPGSGVFGIGPYGPGASAAAAAGIYGPGVFGPYGPGISAAAAAGPGSGIYGPGASGINGPGSGIYGPGVFGPGISAAAAAGIYVFGPGVFGPYGPGASAAAAAGIYGSGPGVFGPYGPGISGSGVFGPGVFGPYASAAAAAGPGSGVFGPGAS

SEQ ID NO: 41 - protein, 590 aa, Artificial Sequence
  Met-PRT917
MGPGLIGPYGPGASAAAAAGVNGPGSGLIGPGVSGVYGPGLIGPGLIGPGSSAAAAAGPGVYGPGLIGPSASAAAAAGPGSGLIGPGASGVYGPGLIGPGLIGPGSSAAAAAGVYGSGPGLIGPYGSAAAAAGPGSGVYGVGPYGPGASGPGVYGPGLIGPSASAAAAAGSGLIGPGVYGPYASAAAAAGVYGSGPGLIGPYGPGVSGSGLIGPGLIGPYASAAAAAGPGLIGPYGPGSSAAAAAGVYGYGPGLIGPYGPGASGVNGPGSGVYGPGLIGPGVSAAAAAGPGLIGPYGPGASAAAAAGVYGPGLIGPGVYGPGSSGPGLIGPYGPGSSAAAAAGVYGPGLIGPYGPGVSAAAAAGVYLIGPGLIGPYGPGASGPGLIGPYGPGASAAAAAGPGVYGPGLIGPSASAAAAAGVYGSGPGVYGPYGPGVSGPGSGLIGVGPYGPGASAAAAAGVYGPGLIGPYGPGVSAAAAAGPGSGVYGPGASGVNGPGSGVYGPGLIGPGVSAAAAAGVYLIGPGLIGPYGPGASAAAAAGVYGSGPGLIGPYGPGVSGSGLIGPGLIGPYASAAAAAGPGSGLIGPGAS

SEQ ID NO: 42 - protein, 587 aa, Artificial Sequence
  Met-PRT1028
MGPGIFGPYGPGASAAAAAGTGPGSGIFGPGTSGTYGPGIFGPGIFGPGSSAAAAAGPGTYGPGIFGPSASAAAAAGPGSGIFGPGASGTYGPGIFGPGIFGPGSSAAAAAGTYGSGPGIFGPYGSAAAAAGPGSGTYGTGPYGPGASGPGTYGPGIFGPSASAAAAAGSGIFGPGTYGPYASAAAAAGTYGSGPGIFGPYGPGTSGSGIFGPGIFGPYASAAAAAGPGIFGPYGPGSSAAAAAGTYGYGPGIFGPYGPGASGTGPGSGTYGPGIFGPGTSAAAAAGPGIFGPYGPGASAAAAAGTYGPGIFGPGTYGPGSSGPGIFGPYGPGSSAAAAAGTYGPGIFGPYGPGTSAAAAAGTYIFGPGIFGPYGPGASGPGIFGPYGPGASAAAAAGPGTYGPGIFGPSASAAAAAGTYGSGPGTYGPYGPGTSGPGSGIFGTGPYGPGASAAAAAGTYGPGIFGPYGPGTSAAAAAGPGSGTYGPGASGTGPGSGTYGPGIFGPGTSAAAAAGTYIFGPGIFGPYGPGASAAAAAGTYGSGPGIFGPYGPGTSGSGIFGPGIFGPYASAAAAAGPGSGIFGPGAS

SEQ ID NO: 43 - protein, 601 aa, Artificial Sequence
  PRT917
MHHHHHHSSGSSGPGLIGPYGPGASAAAAAGVNGPGSGLIGPGVSGVYGPGLIGPGLIGPGSSAAAAAGPGVYGPGLIGPSASAAAAAGPGSGLIGPGASGVYGPGLIGPGLIGPGSSAAAAAGVYGSGPGLIGPYGSAAAAAGPGSGVYGVGPYGPGASGPGVYGPGLIGPSASAAAAAGSGLIGPGVYGPYASAAAAAGVYGSGPGLIGPYGPGVSGSGLIGPGLIGPYASAAAAAGPGLIGPYGPGSSAAAAAGVYGYGPGLIGPYGPGASGVNGPGSGVYGPGLIGPGVSAAAAAGPGLIGPYGPGASAAAAAGVYGPGLIGPGVYGPGSSGPGLIGPYGPGSSAAAAAGVYGPGLIGPYGPGVSAAAAAGVYLIGPGLIGPYGPGASGPGLIGPYGPGASAAAAAGPGVYGPGLIGPSASAAAAAGVYGSGPGVYGPYGPGVSGPGSGLIGVGPYGPGASAAAAAGVYGPGLIGPYGPGVSAAAAAGPGSGVYGPGASGVNGPGSGVYGPGLIGPGVSAAAAAGVYLIGPGLIGPYGPGASAAAAAGVYGSGPGLIGPYGPGVSGSGLIGPGLIGPYASAAAAAGPGSGLIGPGAS

SEQ ID NO: 44 - protein, 598 aa, Artificial Sequence
  PRT1028
MHHHHHHSSGSSGPGIFGPYGPGASAAAAAGTGPGSGIFGPGTSGTYGPGIFGPGIFGPGSSAAAAAGPGTYGPGIFGPSASAAAAAGPGSGIFGPGASGTYGPGIFGPGIFGPGSSAAAAAGTYGSGPGIFGPYGSAAAAAGPGSGTYGTGPYGPGASGPGTYGPGIFGPSASAAAAAGSGIFGPGTYGPYASAAAAAGTYGSGPGIFGPYGPGTSGSGIFGPGIFGPYASAAAAAGPGIFGPYGPGSSAAAAAGTYGYGPGIFGPYGPGASGTGPGSGTYGPGIFGPGTSAAAAAGPGIFGPYGPGASAAAAAGTYGPGIFGPGTYGPGSSGPGIFGPYGPGSSAAAAAGTYGPGIFGPYGPGTSAAAAAGTYIFGPGIFGPYGPGASGPGIFGPYGPGASAAAAAGPGTYGPGIFGPSASAAAAAGTYGSGPGTYGPYGPGTSGPGSGIFGTGPYGPGASAAAAAGTYGPGIFGPYGPGTSAAAAAGPGSGTYGPGASGTGPGSGTYGPGIFGPGTSAAAAAGTYIFGPGIFGPYGPGASAAAAAGTYGSGPGIFGPYGPGTSGSGIFGPGIFGPYASAAAAAGPGSGIFGPGAS

SEQ ID NO: 45 - protein, 605 aa, Artificial Sequence
  PRT#1001,CRY1_L_A5_giza_QtoVFI_Cys4
MHHHHHHSSGSSCGPGVFGPYGPGASAAAAAGINGPGSGVFGPGISCGIYGPGVFGPGVFGPGSSAAAAAGPGIYGPGVFGPSASAAAAAGPGSGVFGPGASGIYGPGVFGPGVFGPGSSAAAAAGIYGSGPGVFGPYGSAAAAAGPGSGIYGIGPYGPGASGPGIYGPGVFGPSASAAAAAGSGVFGPGIYGPYASAAAAAGIYGSGPGVFGPYGPGISGSGVFGPGVFGPYASAAAAAGPGVFGPYGPGSSAAAAAGIYGYGPGVFGPYGPGASGINGPGSGIYGPGVFGPGISAAAAAGPGVFGPYGPGASAAAAAGIYGPGVFGPGIYGPGSSGPGVFGPYGPGSSAAAAAGIYGPGVFGPYGPGISAAAAAGIYVFGPGVFGPYGPGASGPGVFGPYGPGASAAAAAGPGIYGPGVFGPSASAAAAAGIYGSGPGIYGPYGPGISGPGSGVFGIGPYGPGASAAAAAGIYGPGVFGPYGPGISAAAAAGPGSGIYGPGASGINGPGSGIYGPGVFGPGISAAAAAGIYVFGPGVFGPYGPGASAAAAAGIYGSGPGVFGPYGPGISGCSGVFGPGVFGPYASAAAAAGPGCSGVFGPGAS

SEQ ID NO: 46 - protein, 1180 aa, Artificial Sequence
  PRT1
MCGPGVFGPYGPGASAAAAAGINGPGSGVFGPGISGIYGPGVFGPGVFGPGSSAAAAAGPGIYGPGVFGPSASAAAAAGPGSGVFGPGASGIYGPGVFGPGVFGPGSSAAAAAGIYGSGPGVFGPYGSAAAAAGPGSGIYGIGPYGPGASGPGIYGPGVFGPSASAAAAAGSGVFGPGIYGPYASAAAAAGIYGSGPGVFGPYGPGISGSGVFGPGVFGPYASAAAAAGPGVFGPYGPGSSAAAAAGIYGYGPGVFGPYGPGASGINGPGSGIYGPGVFGPGISAAAAAGPGVFGPYGPGASAAAAAGIYGPGVFGPGIYGPGSSGPGVFGPYGPGSSAAAAAGIYGPGVFGPYGPGISAAAAAGIYVFGPGVFGPYGPGASGPGVFGPYGPGASAAAAAGPGIYGPGVFGPSASAAAAAGIYGSGPGIYGPYGPGISGPGSGVFGIGPYGPGASAAAAAGIYGPGVFGPYGPGISAAAAAGPGSGIYGPGASGINGPGSGIYGPGVFGPGISAAAAAGIYVFGPGVFGPYGPGASAAAAAGIYGSGPGVFGPYGPGISGSGVFGPGVFGPYASAAAAAGPGSGVFGPGASGPGVFGPYGPGASAAAAAGINGPGSGVFGPGISGIYGPGVFGPGVFGPGSSAAAAAGPGIYGPGVFGPSASAAAAAGPGSGVFGPGASGIYGPGVFGPGVFGPGSSAAAAAGIYGSGPGVFGPYGSAAAAAGPGSGIYGIGPYGPGASGPGIYGPGVFGPSASAAAAAGSGVFGPGIYGPYASAAAAAGIYGSGPGVFGPYGPGISGSGVFGPGVFGPYASAAAAAGPGVFGPYGPGSSAAAAAGIYGYGPGVFGPYGPGASGINGPGSGIYGPGVFGPGISAAAAAGPGVFGPYGPGASAAAAAGIYGPGVFGPGIYGPGSSGPGVFGPYGPGSSAAAAAGIYGPGVFGPYGPGISAAAAAGIYVFGPGVFGPYGPGASGPGVFGPYGPGASAAAAAGPGIYGPGVFGPSASAAAAAGIYGSGPGIYGPYGPGISGPGSGVFGIGPYGPGASAAAAAGIYGPGVFGPYGPGISAAAAAGPGSGIYGPGASGINGPGSGIYGPGVFGPGISAAAAAGIYVFGPGVFGPYGPGASAAAAAGIYGSGPGVFGPYGPGISGSGVFGPGVFGPYASAAAAAGPGSGVFGPGAS

SEQ ID NO: 47 - protein, 591 aa, Artificial Sequence
  PRT2
MCGPGVFGPYGPGASAAAAAGINGPGSGVFGPGISGIYGPGVFGPGVFGPGSSAAAAAGPGIYGPGVFGPSASAAAAAGPGSGVFGPGASGIYGPGVFGPGVFGPGSSAAAAAGIYGSGPGVFGPYGSAAAAAGPGSGIYGIGPYGPGASGPGIYGPGVFGPSASAAAAAGSGVFGPGIYGPYASAAAAAGIYGSGPGVFGPYGPGISGSGVFGPGVFGPYASAAAAAGPGVFGPYGPGSSAAAAAGIYGYGPGVFGPYGPGASGINGPGSGIYGPGVFGPGISAAAAAGPGVFGPYGPGASAAAAAGIYGPGVFGPGIYGPGSSGPGVFGPYGPGSSAAAAAGIYGPGVFGPYGPGISAAAAAGIYVFGPGVFGPYGPGASGPGVFGPYGPGASAAAAAGPGIYGPGVFGPSASAAAAAGIYGSGPGIYGPYGPGISGPGSGVFGIGPYGPGASAAAAAGIYGPGVFGPYGPGISAAAAAGPGSGIYGPGASGINGPGSGIYGPGVFGPGISAAAAAGIYVFGPGVFGPYGPGASAAAAAGIYGSGPGVFGPYGPGISGSGVFGPGVFGPYASAAAAAGPGSGVFGPGAS

SEQ ID NO: 48 - protein, 592 aa, Artificial Sequence
  PRT3
MCGPGVFGPYGPGASAAAAAGINGPGSGVFGPGISGIYGPGVFGPGVFGPGSSAAAAAGPGIYGPGVFGPSASAAAAAGPGSGVFGPGASGIYGPGVFGPGVFGPGSSAAAAAGIYGSGPGVFGPYGSAAAAAGPGSGIYGIGPYGPGASGPGIYGPGVFGPSASAAAAAGSGVFGPGIYGPYASAAAAAGIYGSGPGVFGPYGPGISGSGVFGPGVFGPYASAAAAAGPGVFGPYGPGSSAAAAAGIYGYGPGVFGPYGPGASGINGPGSGIYGPGVFGPGISAAAAAGPGVFGPYGPGASAAAAAGIYGPGVFGPGIYGPGSSGPGVFGPYGPGSSAAAAAGIYGPGVFGPYGPGISAAAAAGIYVFGPGVFGPYGPGASGPGVFGPYGPGASAAAAAGPGIYGPGVFGPSASAAAAAGIYGSGPGIYGPYGPGISGPGSGVFGIGPYGPGASAAAAAGIYGPGVFGPYGPGISAAAAAGPGSGIYGPGASGINGPGSGIYGPGVFGPGISAAAAAGIYVFGPGVFGPYGPGASAAAAAGIYGSGPGVFGPYGPGISGSGVFGPGVFGPYASAAAAAGPGSGVFGPGASC

SEQ ID NO: 49 - protein, 594 aa, Artificial Sequence
  PRT4
MCGPGVFGPYGPGASAAAAAGINGPGSGVFGPGISCGIYGPGVFGPGVFGPGSSAAAAAGPGIYGPGVFGPSASAAAAAGPGSGVFGPGASGIYGPGVFGPGVFGPGSSAAAAAGIYGSGPGVFGPYGSAAAAAGPGSGIYGIGPYGPGASGPGIYGPGVFGPSASAAAAAGSGVFGPGIYGPYASAAAAAGIYGSGPGVFGPYGPGISGSGVFGPGVFGPYASAAAAAGPGVFGPYGPGSSAAAAAGIYGYGPGVFGPYGPGASGINGPGSGIYGPGVFGPGISAAAAAGPGVFGPYGPGASAAAAAGIYGPGVFGPGIYGPGSSGPGVFGPYGPGSSAAAAAGIYGPGVFGPYGPGISAAAAAGIYVFGPGVFGPYGPGASGPGVFGPYGPGASAAAAAGPGIYGPGVFGPSASAAAAAGIYGSGPGIYGPYGPGISGPGSGVFGIGPYGPGASAAAAAGIYGPGVFGPYGPGISAAAAAGPGSGIYGPGASGINGPGSGIYGPGVFGPGISAAAAAGIYVFGPGVFGPYGPGASAAAAAGIYGSGPGVFGPYGPGISGCSGVFGPGVFGPYASAAAAAGPGCSGVFGPGAS

SEQ ID NO: 50 - protein, 598 aa, Artificial Sequence
  PRT5
MCGPGVFGPYGPGASAAAAAGINGPGSGVFGPGISCGIYGPGVFGPGVFGPGSSAAAAAGPGIYGPGCVFGPSASAAAAAGPGSGVFGPGASCGIYGPGVFGPGVFGPGSSAAAAAGIYGSGPGVFGPYGSAAAAAGPGSGIYGIGPYGPGASGPGIYGPGVFGPSASAAAAAGSGVFGPGIYGPYASAAAAAGIYGSGPGVFGPYGPGISGSGVFGPGVFGPYASAAAAAGPGVFGPYGPGSSAAAAAGIYGYGPGVFGPYGPGASGINGPGSGIYGPGVFGPGISAAAAAGPGVFGPYGPGASAAAAAGIYGPGVFGPGIYGPGSSGPGVFGPYGPGSSAAAAAGIYGPGVFGPYGPGISAAAAAGIYVFGPGVFGPYGPGASGPGVFGPYGPGASAAAAAGPGIYGPGVFGPSASAAAAAGIYGSGPGIYGPYGPGISGPGSGVFGIGPYGPGASAAAAAGIYGPGVFGPYGPGISAAAAAGPGSGIYGPGASGINGPGCSGIYGPGVFGPGISAAAAAGIYVFGPGCVFGPYGPGASAAAAAGIYGSGPGVFGPYGPGISGCSGVFGPGVFGPYASAAAAAGPGCSGVFGPGAS

SEQ ID NO: 51 - protein, 606 aa, Artificial Sequence
  PRT6
MCGPGVFGPYGPGASAAAAAGINGPGSGVFGPGISCGIYGPGVFGPGVFGPGSSAAAAAGPGIYGPGCVFGPSASAAAAAGPGSGVFGPGASCGIYGPGVFGPGVFGPGSSAAAAAGIYGSGPGCVFGPYGSAAAAAGPGSGIYGIGPYGPGASCGPGIYGPGVFGPSASAAAAAGSGVFGPGCIYGPYASAAAAAGIYGSGPGVFGPYGPGISGCSGVFGPGVFGPYASAAAAAGPGVFGPYGPGSSAAAAAGIYGYGPGVFGPYGPGASGINGPGSGIYGPGVFGPGISAAAAAGPGVFGPYGPGASAAAAAGIYGPGVFGPGIYGPGSSGPGVFGPYGPGSSAAAAAGIYGPGVFGPYGPGISAAAAAGIYVFGPGVFGPYGPGASCGPGVFGPYGPGASAAAAAGPGIYGPGCVFGPSASAAAAAGIYGSGPGIYGPYGPGISGPGCSGVFGIGPYGPGASAAAAAGIYGPGVFCGPYGPGISAAAAAGPGSGIYGPGASGINGPGCSGIYGPGVFGPGISAAAAAGIYVFGPGCVFGPYGPGASAAAAAGIYGSGPGVFGPYGPGISGCSGVFGPGVFGPYASAAAAAGPGCSGVFGPGAS

SEQ ID NO: 52 - protein, 592 aa, Artificial Sequence
  PRT7
MCGPGQQGPYGPGASAAAAAGQNGPGSGQQGPGQSGQYGPGQQGPGQQGPGSSAAAAAGPGQYGPGQQGPSASAAAAAGPGSGQQGPGASGQYGPGQQGPGQQGPGSSAAAAAGQYGSGPGQQGPYGSAAAAAGPGSGQYGQGPYGPGASGPGQYGPGQQGPSASAAAAAGSGQQGPGQYGPYASAAAAAGQYGSGPGQQGPYGPGQSGSGQQGPGQQGPYASAAAAAGPGQQGPYGPGSSAAAAAGQYGYGPGQQGPYGPGASGQNGPGSGQYGPGQQGPGQSAAAAAGPGQQGPYGPGASAAAAAGQYGPGQQGPGQYGPGSSGPGQQGPYGPGSSAAAAAGQYGPGQQGPYGPGQSAAAAAGQYQQGPGQQGPYGPGASGPGQQGPYGPGASAAAAAGPGQYGPGQQGPSASAAAAAGQYGSGPGQYGPYGPGQSGPGSGQQGQGPYGPGASAAAAAGQYGPGQQGPYGPGQSAAAAAGPGSGQYGPGASGQNGPGSGQYGPGQQGPGQSAAAAAGQYQQGPGQQGPYGPGASAAAAAGQYGSGPGQQGPYGPGQSGSGQQGPGQQGPYASAAAAAGPGSGQQGPGASC

SEQ ID NO: 53 - protein, 592 aa, Artificial Sequence
  PRT8
MCGPGQQGPYGPGASAAAAAGQNGPGSGQQGPGQSGQYGPGQQGPGQQGPGSSAAAAAGPGQYGPGQQGPSASAAAAAGPGSGQQGPGASGQYGPGQQGPGQQGPGSSAAAAAGQYGSGPGQQGPYGSAAAAAGPGSGQYGQGPYGPGASGPGQYGPGQQGPSASAAAAAGSGQQGPGQYGPYASAAAAAGQYGSGPGQQGPYGPGQSGSGQQGPGQQGPYASAAAAAGPGQQGPYGPGSSAAAAAGQYGYGPGQQGPYGPGASGQNGPGSGQYGPGQQGPGQSAAAAAGPGQQGPYGPGASAAAAAGQYGPGQQGPGQYGPGSSGPGQQGPYGPGSSAAAAAGQYGPGQQGPYGPGQSAAAAAGQYQQGPGQQGPYGPGASGPGQQGPYGPGASAAAAAGPGQYGPGQQGPSASAAAAAGQYGSGPGQYGPYGPGQSGPGSGQQGQGPYGPGASAAAAAGQYGPGQQGPYGPGQSAAAAAGPGSGQYGPGASGQNGPGSGQYGPGQQGPGQSAAAAAGQYQQGPGQQGPYGPGASAAAAAGQYGSGPGQQGPYGPGQSGSGQQGPGQQGPYASAAAAAGPGSGCQQGPGAS

SEQ ID NO: 54 - protein, 598 aa, Artificial Sequence
  PRT9
MCGPGQQGPYGPGASAAAAAGQNGPGSGQQGPGQSCGQYGPGQQGPGQQGPGSSAAAAAGPGQYGPGQQCGPSASAAAAAGPGSGQQGPGASGQYCGPGQQGPGQQGPGSSAAAAAGQYGSGPGQQGPYGSAAAAAGPGSGQYGQGPYGPGASGPGQYGPGQQGPSASAAAAAGSGQQGPGQYGPYASAAAAAGQYGSGPGQQGPYGPGQSGSGQQGPGQQGPYASAAAAAGPGQQGPYGPGSSAAAAAGQYGYGPGQQGPYGPGASGQNGPGSGQYGPGQQGPGQSAAAAAGPGQQGPYGPGASAAAAAGQYGPGQQGPGQYGPGSSGPGQQGPYGPGSSAAAAAGQYGPGQQGPYGPGQSAAAAAGQYQQGPGQQGPYGPGASGPGQQGPYGPGASAAAAAGPGQYGPGQQGPSASAAAAAGQYGSGPGQYGPYGPGQSGPGSGQQGQGPYGPGASAAAAAGQYGPGQQGPYGPGQSAAAAAGPGSGQYGPGASGQNGPGCSGQYGPGQQGPGQSAAAAAGQYQQGPGQQCGPYGPGASAAAAAGQYGSGPGQQGPYGPGQSCGSGQQGPGQQGPYASAAAAAGPGSGCQQGPGAS

SEQ ID NO: 55 - protein, 606 aa, Artificial Sequence
  PRT10
MCGPGQQGPYGPGASAAAAAGQNGPGSGQQGPGQSCGQYGPGQQGPGQQGPGSSAAAAAGPGQYGPGQQCGPSASAAAAAGPGSGQQGPGASGQYCGPGQQGPGQQGPGSSAAAAAGQYGSCGPGQQGPYGSAAAAAGPGSGQYGQGPYGPGASCGPGQYGPGQQGPSASAAAAAGSGQQGPGCQYGPYASAAAAAGQYGSGPGQQGPYGPGQSGCSGQQGPGQQGPYASAAAAAGPGQQGPYGPGSSAAAAAGQYGYGPGQQGPYGPGASGQNGPGSGQYGPGQQGPGQSAAAAAGPGQQGPYGPGASAAAAAGQYGPGQQGPGQYGPGSSGPGQQGPYGPGSSAAAAAGQYGPGQQGPYGPGQSAAAAAGQYQQGPGQQGPYGPGACSGPGQQGPYGPGASAAAAAGPGQYGPGQQCGPSASAAAAAGQYGSGPGQYGPYGPGQSCGPGSGQQGQGPYGPGASAAAAAGQYGPGQQCGPYGPGQSAAAAAGPGSGQYGPGASGQNGPGCSGQYGPGQQGPGQSAAAAAGQYQQGPGQQCGPYGPGASAAAAAGQYGSGPGQQGPYGPGQSCGSGQQGPGQQGPYASAAAAAGPGSGCQQGPGAS

SEQ ID NO: 56 - protein, 1179 aa, Artificial Sequence; identical to SEQ ID NO: 32
  PRT11

SEQ ID NO: 57 - protein, 590 aa, Artificial Sequence; identical to SEQ ID NO: 29
  PRT12

SEQ ID NO: 58 - protein, 590 aa, Artificial Sequence; identical to SEQ ID NO: 7
  PRT13

SEQ ID NO: 59 - protein, 590 aa, Artificial Sequence; identical to SEQ ID NO: 7
  PRT14

SEQ ID NO: 60 - protein, 1191 aa, Artificial Sequence
  PRT15
MHHHHHHSSGSSCGPGVFGPYGPGASAAAAAGINGPGSGVFGPGISGIYGPGVFGPGVFGPGSSAAAAAGPGIYGPGVFGPSASAAAAAGPGSGVFGPGASGIYGPGVFGPGVFGPGSSAAAAAGIYGSGPGVFGPYGSAAAAAGPGSGIYGIGPYGPGASGPGIYGPGVFGPSASAAAAAGSGVFGPGIYGPYASAAAAAGIYGSGPGVFGPYGPGISGSGVFGPGVFGPYASAAAAAGPGVFGPYGPGSSAAAAAGIYGYGPGVFGPYGPGASGINGPGSGIYGPGVFGPGISAAAAAGPGVFGPYGPGASAAAAAGIYGPGVFGPGIYGPGSSGPGVFGPYGPGSSAAAAAGIYGPGVFGPYGPGISAAAAAGIYVFGPGVFGPYGPGASGPGVFGPYGPGASAAAAAGPGIYGPGVFGPSASAAAAAGIYGSGPGIYGPYGPGISGPGSGVFGIGPYGPGASAAAAAGIYGPGVFGPYGPGISAAAAAGPGSGIYGPGASGINGPGSGIYGPGVFGPGISAAAAAGIYVFGPGVFGPYGPGASAAAAAGIYGSGPGVFGPYGPGISGSGVFGPGVFGPYASAAAAAGPGSGVFGPGASGPGVFGPYGPGASAAAAAGINGPGSGVFGPGISGIYGPGVFGPGVFGPGSSAAAAAGPGIYGPGVFGPSASAAAAAGPGSGVFGPGASGIYGPGVFGPGVFGPGSSAAAAAGIYGSGPGVFGPYGSAAAAAGPGSGIYGIGPYGPGASGPGIYGPGVFGPSASAAAAAGSGVFGPGIYGPYASAAAAAGIYGSGPGVFGPYGPGISGSGVFGPGVFGPYASAAAAAGPGVFGPYGPGSSAAAAAGIYGYGPGVFGPYGPGASGINGPGSGIYGPGVFGPGISAAAAAGPGVFGPYGPGASAAAAAGIYGPGVFGPGIYGPGSSGPGVFGPYGPGSSAAAAAGIYGPGVFGPYGPGISAAAAAGIYVFGPGVFGPYGPGASGPGVFGPYGPGASAAAAAGPGIYGPGVFGPSASAAAAAGIYGSGPGIYGPYGPGISGPGSGVFGIGPYGPGASAAAAAGIYGPGVFGPYGPGISAAAAAGPGSGIYGPGASGINGPGSGIYGPGVFGPGISAAAAAGIYVFGPGVFGPYGPGASAAAAAGIYGSGPGVFGPYGPGISGSGVFGPGVFGPYASAAAAAGPGSGVFGPGAS

SEQ ID NO: 61 - protein, 602 aa, Artificial Sequence
  PRT16
MHHHHHHSSGSSCGPGVFGPYGPGASAAAAAGINGPGSGVFGPGISGIYGPGVFGPGVFGPGSSAAAAAGPGIYGPGVFGPSASAAAAAGPGSGVFGPGASGIYGPGVFGPGVFGPGSSAAAAAGIYGSGPGVFGPYGSAAAAAGPGSGIYGIGPYGPGASGPGIYGPGVFGPSASAAAAAGSGVFGPGIYGPYASAAAAAGIYGSGPGVFGPYGPGISGSGVFGPGVFGPYASAAAAAGPGVFGPYGPGSSAAAAAGIYGYGPGVFGPYGPGASGINGPGSGIYGPGVFGPGISAAAAAGPGVFGPYGPGASAAAAAGIYGPGVFGPGIYGPGSSGPGVFGPYGPGSSAAAAAGIYGPGVFGPYGPGISAAAAAGIYVFGPGVFGPYGPGASGPGVFGPYGPGASAAAAAGPGIYGPGVFGPSASAAAAAGIYGSGPGIYGPYGPGISGPGSGVFGIGPYGPGASAAAAAGIYGPGVFGPYGPGISAAAAAGPGSGIYGPGASGINGPGSGIYGPGVFGPGISAAAAAGIYVFGPGVFGPYGPGASAAAAAGIYGSGPGVFGPYGPGISGSGVFGPGVFGPYASAAAAAGPGSGVFGPGAS

SEQ ID NO: 62 - protein, 603 aa, Artificial Sequence
  PRT17
MHHHHHHSSGSSCGPGVFGPYGPGASAAAAAGINGPGSGVFGPGISGIYGPGVFGPGVFGPGSSAAAAAGPGIYGPGVFGPSASAAAAAGPGSGVFGPGASGIYGPGVFGPGVFGPGSSAAAAAGIYGSGPGVFGPYGSAAAAAGPGSGIYGIGPYGPGASGPGIYGPGVFGPSASAAAAAGSGVFGPGIYGPYASAAAAAGIYGSGPGVFGPYGPGISGSGVFGPGVFGPYASAAAAAGPGVFGPYGPGSSAAAAAGIYGYGPGVFGPYGPGASGINGPGSGIYGPGVFGPGISAAAAAGPGVFGPYGPGASAAAAAGIYGPGVFGPGIYGPGSSGPGVFGPYGPGSSAAAAAGIYGPGVFGPYGPGISAAAAAGIYVFGPGVFGPYGPGASGPGVFGPYGPGASAAAAAGPGIYGPGVFGPSASAAAAAGIYGSGPGIYGPYGPGISGPGSGVFGIGPYGPGASAAAAAGIYGPGVFGPYGPGISAAAAAGPGSGIYGPGASGINGPGSGIYGPGVFGPGISAAAAAGIYVFGPGVFGPYGPGASAAAAAGIYGSGPGVFGPYGPGISGSGVFGPGVFGPYASAAAAAGPGSGVFGPGASC

SEQ ID NO: 63 - protein, 605 aa, Artificial Sequence; identical to SEQ ID NO: 45
  PRT18

SEQ ID NO: 64 - protein, 609 aa, Artificial Sequence
  PRT19
MHHHHHHSSGSSCGPGVFGPYGPGASAAAAAGINGPGSGVFGPGISCGIYGPGVFGPGVFGPGSSAAAAAGPGIYGPGCVFGPSASAAAAAGPGSGVFGPGASCGIYGPGVFGPGVFGPGSSAAAAAGIYGSGPGVFGPYGSAAAAAGPGSGIYGIGPYGPGASGPGIYGPGVFGPSASAAAAAGSGVFGPGIYGPYASAAAAAGIYGSGPGVFGPYGPGISGSGVFGPGVFGPYASAAAAAGPGVFGPYGPGSSAAAAAGIYGYGPGVFGPYGPGASGINGPGSGIYGPGVFGPGISAAAAAGPGVFGPYGPGASAAAAAGIYGPGVFGPGIYGPGSSGPGVFGPYGPGSSAAAAAGIYGPGVFGPYGPGISAAAAAGIYVFGPGVFGPYGPGASGPGVFGPYGPGASAAAAAGPGIYGPGVFGPSASAAAAAGIYGSGPGIYGPYGPGISGPGSGVFGIGPYGPGASAAAAAGIYGPGVFGPYGPGISAAAAAGPGSGIYGPGASGINGPGCSGIYGPGVFGPGISAAAAAGIYVFGPGCVFGPYGPGASAAAAAGIYGSGPGVFGPYGPGISGCSGVFGPGVFGPYASAAAAAGPGCSGVFGPGAS

SEQ ID NO: 65 - protein, 617 aa, Artificial Sequence
  PRT20
MHHHHHHSSGSSCGPGVFGPYGPGASAAAAAGINGPGSGVFGPGISCGIYGPGVFGPGVFGPGSSAAAAAGPGIYGPGCVFGPSASAAAAAGPGSGVFGPGASCGIYGPGVFGPGVFGPGSSAAAAAGIYGSGPGCVFGPYGSAAAAAGPGSGIYGIGPYGPGASCGPGIYGPGVFGPSASAAAAAGSGVFGPGCIYGPYASAAAAAGIYGSGPGVFGPYGPGISGCSGVFGPGVFGPYASAAAAAGPGVFGPYGPGSSAAAAAGIYGYGPGVFGPYGPGASGINGPGSGIYGPGVFGPGISAAAAAGPGVFGPYGPGASAAAAAGIYGPGVFGPGIYGPGSSGPGVFGPYGPGSSAAAAAGIYGPGVFGPYGPGISAAAAAGIYVFGPGVFGPYGPGASCGPGVFGPYGPGASAAAAAGPGIYGPGCVFGPSASAAAAAGIYGSGPGIYGPYGPGISGPGCSGVFGIGPYGPGASAAAAAGIYGPGVFCGPYGPGISAAAAAGPGSGIYGPGASGINGPGCSGIYGPGVFGPGISAAAAAGIYVFGPGCVFGPYGPGASAAAAAGIYGSGPGVFGPYGPGISGCSGVFGPGVFGPYASAAAAAGPGCSGVFGPGAS

SEQ ID NO: 66 - protein, 603 aa, Artificial Sequence
  PRT21
MHHHHHHSSGSSCGPGQQGPYGPGASAAAAAGQNGPGSGQQGPGQSGQYGPGQQGPGQQGPGSSAAAAAGPGQYGPGQQGPSASAAAAAGPGSGQQGPGASGQYGPGQQGPGQQGPGSSAAAAAGQYGSGPGQQGPYGSAAAAAGPGSGQYGQGPYGPGASGPGQYGPGQQGPSASAAAAAGSGQQGPGQYGPYASAAAAAGQYGSGPGQQGPYGPGQSGSGQQGPGQQGPYASAAAAAGPGQQGPYGPGSSAAAAAGQYGYGPGQQGPYGPGASGQNGPGSGQYGPGQQGPGQSAAAAAGPGQQGPYGPGASAAAAAGQYGPGQQGPGQYGPGSSGPGQQGPYGPGSSAAAAAGQYGPGQQGPYGPGQSAAAAAGQYQQGPGQQGPYGPGASGPGQQGPYGPGASAAAAAGPGQYGPGQQGPSASAAAAAGQYGSGPGQYGPYGPGQSGPGSGQQGQGPYGPGASAAAAAGQYGPGQQGPYGPGQSAAAAAGPGSGQYGPGASGQNGPGSGQYGPGQQGPGQSAAAAAGQYQQGPGQQGPYGPGASAAAAAGQYGSGPGQQGPYGPGQSGSGQQGPGQQGPYASAAAAAGPGSGQQGPGASC

SEQ ID NO: 67 - protein, 603 aa, Artificial Sequence
  PRT22
MHHHHHHSSGSSCGPGQQGPYGPGASAAAAAGQNGPGSGQQGPGQSGQYGPGQQGPGQQGPGSSAAAAAGPGQYGPGQQGPSASAAAAAGPGSGQQGPGASGQYGPGQQGPGQQGPGSSAAAAAGQYGSGPGQQGPYGSAAAAAGPGSGQYGQGPYGPGASGPGQYGPGQQGPSASAAAAAGSGQQGPGQYGPYASAAAAAGQYGSGPGQQGPYGPGQSGSGQQGPGQQGPYASAAAAAGPGQQGPYGPGSSAAAAAGQYGYGPGQQGPYGPGASGQNGPGSGQYGPGQQGPGQSAAAAAGPGQQGPYGPGASAAAAAGQYGPGQQGPGQYGPGSSGPGQQGPYGPGSSAAAAAGQYGPGQQGPYGPGQSAAAAAGQYQQGPGQQGPYGPGASGPGQQGPYGPGASAAAAAGPGQYGPGQQGPSASAAAAAGQYGSGPGQYGPYGPGQSGPGSGQQGQGPYGPGASAAAAAGQYGPGQQGPYGPGQSAAAAAGPGSGQYGPGASGQNGPGSGQYGPGQQGPGQSAAAAAGQYQQGPGQQGPYGPGASAAAAAGQYGSGPGQQGPYGPGQSGSGQQGPGQQGPYASAAAAAGPGSGCQQGPGAS

SEQ ID NO: 68 - protein, 609 aa, Artificial Sequence
  PRT23
MHHHHHHSSGSSCGPGQQGPYGPGASAAAAAGQNGPGSGQQGPGQSCGQYGPGQQGPGQQGPGSSAAAAAGPGQYGPGQQCGPSASAAAAAGPGSGQQGPGASGQYCGPGQQGPGQQGPGSSAAAAAGQYGSGPGQQGPYGSAAAAAGPGSGQYGQGPYGPGASGPGQYGPGQQGPSASAAAAAGSGQQGPGQYGPYASAAAAAGQYGSGPGQQGPYGPGQSGSGQQGPGQQGPYASAAAAAGPGQQGPYGPGSSAAAAAGQYGYGPGQQGPYGPGASGQNGPGSGQYGPGQQGPGQSAAAAAGPGQQGPYGPGASAAAAAGQYGPGQQGPGQYGPGSSGPGQQGPYGPGSSAAAAAGQYGPGQQGPYGPGQSAAAAAGQYQQGPGQQGPYGPGASGPGQQGPYGPGASAAAAAGPGQYGPGQQGPSASAAAAAGQYGSGPGQYGPYGPGQSGPGSGQQGQGPYGPGASAAAAAGQYGPGQQGPYGPGQSAAAAAGPGSGQYGPGASGQNGPGCSGQYGPGQQGPGQSAAAAAGQYQQGPGQQCGPYGPGASAAAAAGQYGSGPGQQGPYGPGQSCGSGQQGPGQQGPYASAAAAAGPGSGCQQGPGAS

SEQ ID NO: 69 - protein, 617 aa, Artificial Sequence
  PRT24
MHHHHHHSSGSSCGPGQQGPYGPGASAAAAAGQNGPGSGQQGPGQSCGQYGPGQQGPGQQGPGSSAAAAAGPGQYGPGQQCGPSASAAAAAGPGSGQQGPGASGQYCGPGQQGPGQQGPGSSAAAAAGQYGSCGPGQQGPYGSAAAAAGPGSGQYGQGPYGPGASCGPGQYGPGQQGPSASAAAAAGSGQQGPGCQYGPYASAAAAAGQYGSGPGQQGPYGPGQSGCSGQQGPGQQGPYASAAAAAGPGQQGPYGPGSSAAAAAGQYGYGPGQQGPYGPGASGQNGPGSGQYGPGQQGPGQSAAAAAGPGQQGPYGPGASAAAAAGQYGPGQQGPGQYGPGSSGPGQQGPYGPGSSAAAAAGQYGPGQQGPYGPGQSAAAAAGQYQQGPGQQGPYGPGACSGPGQQGPYGPGASAAAAAGPGQYGPGQQCGPSASAAAAAGQYGSGPGQYGPYGPGQSCGPGSGQQGQGPYGPGASAAAAAGQYGPGQQCGPYGPGQSAAAAAGPGSGQYGPGASGQNGPGCSGQYGPGQQGPGQSAAAAAGQYQQGPGQQCGPYGPGASAAAAAGQYGSGPGQQGPYGPGQSCGSGQQGPGQQGPYASAAAAAGPGSGCQQGPGAS

SEQ ID NO: 70 - protein, 12 aa, Artificial Sequence
  HisTag(S)
MHHHHHHSSGSS

SEQ ID NO: 71 - protein, 12 aa, Artificial Sequence
  HisTag(A)
MHHHHHHAAGAA

SEQ ID NO: 72 - protein, 601 aa, Artificial Sequence; identical to SEQ ID NO: 37
  PRT27